European Patent Specification EP 4 259 825 B1, published August 20, 2025. Title: Méthode et kit de détection de Christensenella minuta. Applicant: YSOPIA BIOSCIENCES. The sequence listing filed with the application follows.

SEQUENCE LISTING (14 sequences)

SEQ ID NO: 1 - DNA, 93006 bp, Christensenella minuta
  >CP029256.1:1921147-2014152
atttgtagtgtaaatcagcgtgcggacagtctgtgaacacttgaaatatactatgtagtgtaagtactaatagtatgttacactatgaagagttacaggagcagacaaaggatttcatgatggtactcaaacaaacgcacgagcgccccccaggtgaaggagtttgcttcacgccgagctggagtaaccatagcagtccaaaagccgggatgtacagcatcgcaaaattcacaatatggagctataaggtggatgtggtatagcgtcggaaagtccgaaaatatctgcaaagtgttctgttccggcataaaaaacgcttttcttacgaagaacgtgcggcttatatggttatttttgaattatcctgtgctttttggtagagtcgctataatagtattattattgcagattctcttgaaccgttgaggggcagacattcggcatatagtatttacagagccatattcgacatatgataagaccgcgccgccattgaattcgatatgaaagtatgttaaaaaggaggccagtatgatacagaaaaaaatattgaaaccgtttttatgtcttttatgtattctcgctattcttgcatctgccggatgtggtatgatgggggagctattgaacgttcttgaggaagaaccgaaacccacgaaagagctggaatctacggaagatttaactcagccgagcagagagccgtatactagacgatattattctagcgatgtcgagcgttttgatgtcccgcttggggaacgctccagggagtttttgacaaggatgcttttgtcatcgtattctttgaattcaaggacattatagaagcccaatacactgaagaaaacgaaacgaggcttctcgagctttatgaggaaattaggtccggcctgctggatgttaaaacggacgttagccttgcgaagtatgattattaccttgttatagatgattttttttcgatactttggtgtaaatgtaaatatgatatgatacttacatatccacttgctatgggctaaacttttatccatttgaaaaactcctttcgagtagaatgtagatgttcaggctacatgaaaacgagaaaggagttttttgccctgtaagctttgtttcccacccgtatatagaccgtaccggataaaaaggacagtttccgaaaagccacccccgctgtaggatagaactacaacgggggtgaaaatgtgtatgtcaagaaaatacacacaaatcaaaggatattatgaagaaatggaacgccagcaccaagaaggctgcagctgtcgggaaatcggagaaaagttaggctttacaaaagaacaggtgaaagaatgcctaagaagaccaagacgcaaagcccaaaaacagaacgccagtatcccaaatcggcgtggtcgaccggctaagcaaatgccttgcattctcagtgcattgtaaaaagaggtcaggcagcttcggatggaaaatgaattgctgcgggattttctgaaaacaaccgaaaggaagtgagaacgtctgccaaatatcaggtgatacaaaaatacgcatcgaagtatccaatcattcgcatgtgtgtattctttggggtatcccgcagcggatactacagctttctaaagcggaggatacagccaaaccgggaatccgcattactggggcgaattcaagaatgccgcggcagtggaagatatatgaatacctacggctgtcatcgggtacagatttggatcaaacgccagtacggtgaatactacaattacaagacggtgtggcgtgttatgcacaaatacgggctgctatctaagattcgccgaaagagattctttcattgcggtgagcagatccgtacctaccccaatctattgaatcggaacttccacgccgacaagcctaaccagaaatgggtaacagacatcagttgcatcccaaccagtcagggccccctacctttccatcattcgggatttgtttgatttaagcattgccgcttacaaaacaagtatccatcagagcattaagctggtacttgatatgatacggttggcgatggaaaaagaaacagtcaccgcagagttgcagctccacagtgatcttttctttgcgtttgacatctttgagcgtcttcaataccaagttgatcgattgctctgtgcctgtgcgatgcgctacgatacttaggtcgtaaaggcctcgtatgaccgacaggtacaccgtgccttgttctgtgggggtatatgagtgaaatgaatccggactatcgggaggcgctctatctcacctattttgaggatatgagatatgcgcaggcggcggaggtcacgggaaagacggtgaagcagattaccaacatggtatatcgcggaaaagagagcttgcgcaaactgctggaacgggaggggatcacaaatgcggagtcatgcggaacgggtcgcggataccggcgccgtcgttcccggctcgttcagcttcaagaaatatgaagacggcagagtatacccggacgaaaaccgcatggaaatcctctttacccctgatgatacggaggcatacgccactgcggaatgcactgttaccgtgaccggaataaaatacacaatcacaagcgtcccctacgacatctacatcaacgacaagctgccggggacggcgtttgagaatttagggcttccttccggcatcaacatagaggtcagcaccggcgcgaactttagttccgttcccgtgacatgggacagttcctcctacggcccggactcttatgaggagcagatcattaccggcgatctgcatgttgaaaagagttcatacgcggatcttctggagccgacaagcacagtcaaggctactgccaggataaagctcattgataaccgtgtctttacgcccacgcttgagccgcccacctactccaagcagctctacggaggcgatttgtgcttccttgtcttttctgacaactacctctccggcggaaaggccacggtgaacggcgaaacggttcccggcacgttcaagctggacaaaaatcagaaaatatacggacactcattgacggcgagccagctcctgcaggccgagccgctgcagctgaagggcatcttcactcccaacgaccagaagcggtacaccacggcggaatgtaccgtcggtgtgaatgtcattccccgcagatttgtcaaacccagttacaacagggtgcttaacaacacaaagatcggcatgacctttgaggagctgaacctgtcggagtcgttcagtttcttcgtggttagcgacgaaactccccccggagagctcgagtcgtattctatgaatgttgtcacctcgtgggacgcttcaacttatgaccccaattcgtatgatatgcagacgatctacggtgaagtcgaccgcgccgaattggagaagtatttcaccataccagaggatgccaacctcagggctgtgatcaaggttcagctgcagcccgacccagccgaaacggagatcacgcaggcacccgtattccgctggaaaaacggtgattttacgctgtccgacaacaccatcttctcccagcgaaggtttcaggtgggaacctacaacgcggaagtcggcagtctctttggcggcgtggtaaaggtcaaggggacggataccgtcgtccccggcacattctcatttaagaagggtacgccgctctactcctcgtctccgggcgaatacgacatgacggtggtgttcacgccgacagatccgcgcctccacaagccgacggagaccagcatcaaaataaacgtcatcaaaaacaccctcaaggatgccgatgagccggaacccattaccgataagccgctcggcacgccctttacggagcttgggctgccgaaagatgtggtcgtcaatgccgttgacggcgcttggcgctggattgacgtagcatgggatgcggcgtcctatgacgcggagtccccggattggcagaccatcaccggtacgttggtgtttgatgaatatgacgaaagcacctaccagcagccaggccctgtggtaacggccacgatcagggtaaagctcatcgtcccggattccgcgcctaccgtcaccaccggaaccctgccgacggcttgacgcttaacgcggatacaggcgaaatcagtggcacgcccactgcggcgggcactgcggtctttacggtcaaggtggtcaacgttttgggttcggacacaaaggagctgtcccttgcgatagtcaaggccgagcacaccgccacctttgacggcaacggtggtatgccctctgtcggcagtatgaccaccacgaatcagaagctggtctctctgcccgatgcttcccgcagcaagcacagcttcgacggctggtacaccgaaaagagcggcggcagcgacaacccgcccgtcaccgattatgcgctgcgctttgaaataggaggcggcagccatattgccgacgtgcggggaacgtacaacacctacattgacctgacaaagtacgttccgatccggcgcggctatacctttatcggctggtacagcgaccgcgatctgacaaacaaggtttccggcgtttatctgacgaacgatatgaccgtatatgcaggctggcgcgtgactgcaatcccgcagaccggtgacggcagccaactgggtttgtggagtattacgctatgtgcgtctcttgccggatgtctcgcgctgaccacatggcagctcagacggcgcaagggcgcatcacgggaaactgcagaaaagtaatcagcacacctttgtggcacgggtttgttcccccgtgccacattcgctatcttcccaggaaaaagacggctgtccttttgaagaacagccgtcctgcttttactgttgatgtgtatgcacctggatatcattcctcaaacaggtacaggagatagccgtacccatcggactccatctttgcataaggcacaaagcggagggacgcactgttgatgcagtagcgcacgccgttgggcgattccggatcaccggtaaatacatgaccgagatgagagtctccagcgcggcttctgacctccgtgcggcgcataccatggctcaggtcctccagctccaccacggcaggctcctcaatgggcttggtaaaggcgggccagccgcagccgctctcgaacttgtccgtggaggaaaagagcggttcgccggtaacgatgtccacatagatgcctttctcgaactggttccagaactcattgctgaagggacgctccgtgccgctctcctgggtgacccggtactgctccgccgtcagcttgtcccggacggactccgccgcgggcttttggtagtcgcccggatcgatgcgcagcttggagaacagctccatctccgcttttgggatatggcagtagccgttcggattcttctccagatagtcctggtggtactcctcggcgggatagtagtttttcagcgggccgatctccacgaagaacttctcgctgcgtccccgctcaatctcggcgatgcgttccaccgtctccttcgcgctttcgttagtgtagtagacgccggtctggtactggctcccgatgtcgttgccctgccggttttctaccgtagggtcggtgacgtagaagtaggccagcagcagggcgtcgagacttatctgctcggggtcgtattccacccgcacggtctcccggaagccggtgttccccttgcagacggtctgatagtcggcgtccgcctcgcaggtaccgttggcgtagccgctctcggcatccagaacgccggggatggactgcatcagctgttccagtccccaaaagcagccgcctgccagatagatgacattttccgtggtatccataaacatgctctcctcgccggacatatcagagggatgcccggccatttccttcgattccgttttctgcggcatattcttatgtgctgcggcgcagccgctcagtagcagtgccgcagcaagcagaagcggtaatactctccgatacatggtggtttcctcctttctactacaataatttatggataggatatggcagccagccatacgcctttccatcccatagtctaagctacaataaggggagtaattggtctgacgactcctttcttgggtctacacgcccgtacgtgagacagtcagccatcctcttgttgcagcgttcgttttgcaggtagagccaccactcgtgcgttcgtgtcactcagtagattgaataggcaatgggtaagagatgggcaccgattacaatacatcaatcaggaggaatacttatgaacgctgtcggtatcgacatttccaaaggcaagtgcatggttgctatcctgcgtcccttcggtgaggtggttgcttcaccttttgaaattcagcacaccgctcatgaactcagacgtttggttgaacgtctgaaaagtttggacggtgaaacccgcattgttatggagcatactggcaattactatctgcctgtcgccaggcatctgcacgaagccggcctctatgtgtccgttgtcaatgctattcttgtacatgactacggtcaaaattcccttagacgggtcaaaacggacaagatagatgctgttaaaatcgccagctatgctctaagccattggcttgatcttccgcaatatgcgccggaagaagacgttcgccacatgcttaaaacctgcgcccgccagtgcaaccagtacgttaagcagagtgttatgcttaaaaacagcctcatcgctttgcttgaccaaacctttccgagtgtcaacatgctgttctccagcccgccccgcaagggggacggtcacgaaaaatggattgacttcgtgggtaaattttggcattttgaatgcgtcaacagcctttccaaaaacgtttttacccagcgctatcaaaaatggtgcaaaagaacaggttacaactttctttccactaaggccgctgccatctacgatttcgcctgcatacaagtcagtacactgcctcgaagcacctttgccaaacagcttattactcaagctgtgtcgcagcttaactccctatcggaaacgctggctctgattcggcagcagatgctttcccttgcctccggcttgccggaatttcctgttgtcatggctatgcaaggggtcggcaatgtgttaggacctcaactcatggctgaaattggcgatgtgcgacgtttcaaccgtaagcagtcgctggttgcttttgccggtatcgacgcaccgcctttccagtccggcgcctttgaagcacagagtaccggcatttccaaacgaggttcttcctcactcagaaagacgctttttcaggtcatggactgcctgctcaaacacgcgccctctcatgatgctgtattccaatatcttgacaaaaaacgcggcgagggtaagcattattacgtctacatgatggcaggagccaacaagttcctgcgtatctactacgcacgggttaaggagcatctaggcagtttggcggttcagtagcccacatattctttttgcttggcttaccagcttatttcagggtggttttatttgatgttccattttttacctttcattttttattcatttccggcttgacttttctttgcaggtctgaggagataaattcgcttgtcagcccatatcggcggcaagagcctggtcgatgagcttttgcagcgtctccgcctgctttttttccgtgacggcacctgtgatgggctctcccacgatgttgccgttgcggtcaaccacataggtggtgggataagcaaagatgttcgtggtaaactttcccgcctcgccgtcggaagcgaaatacacattctgataagtcgcgcctttcttggcgagtacatctttcgcctcagaaattgccgctttgtcgccgtccagtgtgaaggtgttgacaccgatgagcgcgccgcccttctcagtaagctccttgttcagcgcatccaactcggcaagctcgcccacgcagggattgcaggtggtaaaccaaaaattcactacggtgacggcgttgccggagaatagctcatcgctcttcaccgcgttcccatccaagtctttaccctcaaatgcagggaacttctgcatactgccgtcatcgggcggcgtggtcatgtcgctgcccgcaggcatactcatggttccatccatggattgctgtgccgcctcggggtattttttctcaatcatggtcagcttgttttcgatgtcgcggattttctccgcttcttcctgaagcagtttcagctcatccgccgtaaactgatccttggcggattcgattgtactgagcaggaaatcaccgtagtttttgccgtcttcctgcatggtcatgcccttgtcggccgccatgaataccttttcccaaagcgctgtgttctccgagagaatggcattttcctgtgccagcagatctttgtgcatggcagccgcttcctcggcgttcttcggctcattgctcatcccatccattttgtcgccgccctttgcgccgcaggctgccagagacagcaccatcagtgcgagaagcaacagcgccagcaatcggccggcagtattcattctattcatccgttttgttcctccttgttattgttgtttttctgcggctgttctgccgcctttgttttatctttaccgtttccgaagccgtagcggaagcacacggcgttggtcggacaggctcggacgcacatcccgcagcgaatgcactctgtatggttgggcgtctttgtcacatccacatccattttgcaggctctggcgcattttccgcaggagacgcacttgtttttgtccaccttcatctggaacagggacaccctgttgaacagcgcgtagaacgcgcccagcgggcagagccacttgcagaagggacggtagaatacgatactcagcgcaatcaccgccagcaggatgctgaacttccatgtaaacaggctgcccagcgccgcccgaatgccggaattggcaagggacagcggaatggccccctccagcacgccctgcgggcagaggtatttgcagaagaaagggtcgcccatgcccacatcgttcacaaggaatgccggcagcagcaaaaccatcaccagcaaaacggcgtacttgaggtatcgcagcggcttcagccttttcgtggacagcttcttcgtgggaatcttgtgcagcagctcctgaaaccagccgaagggacacagaaaaccgcagataaagcgtcccagcaggactcccagcaaaatgaggaagcctgtgatataataggagaagctgaacttggaagaccctaccaccgcctgaaacgccccgatggggcaagcgccggaggccgccgggcaggagtagcagttcaaccccggcacacagacggttttccctgcgccctgatacagtccacccctgaggaaattcggcaggtgcaggttggtcaataaagttgcccccgcctgtatccagccccggaagcgggacatagtctgtgacacgcccgaaaacttcttacccaatgcccacacactccagacataatttgattgctttgctcagcaccgccgccgcctcgccgcgccatacgccgaagcacagcatggcgattcccgcaaccagcagcaaggcctgcgccgcagtcttttttacatgactcaattccatcaccctttcgttttttctgccaccatcataacgcgagaaagttaaaatccctgttaagaacgaaaatttaacgcaaaccttatctgtttttgctataatttaagaacaacatgaaaatgaagaataaaaaggagggctctcatgcaccttttagtaattgaagatgaacgcgccctgtgcgagaccatcgtccgcagcctgcggcggctggcctacagcgtagattactgctacgacggggagaaggcgctggagctgatcgccgttgaaaaatacgatctcatcctgctggatctgaacctgccggggaaggacggcatgacggtgctgcgcaccctgcggcagacagaccgggagacgagggtgctgatcctctccgcccgcagcgaggtggaggacaaggtggaggggctggatgcgggcgccaacgactatctggcaaagccctttcacttagccgagctggaggcccgcattcgcagcctgactctgcggcagttcacccagcaggatgtgctgttgacctgcggagccttgacctttgacacgcgctcccgcaccgcttccgtcaacgggcagacattgacgctgacccgcaaggaaacgggcattctggaatatctgatggtgcaccaggggcggcctgtgagtcaggaggagctgatggatcatgtctgggacaacagcgtggacagcttcagcaactccattcgggtacatatctccgccctgcgcaaaaagctccgggtcgccctgggttacgaccccatccgcaaccgtatcggcgagggctatctgatgggaggcgaggagacatgaggaagatatctttgaaatggcgcatcaccctgatgaccgtcctgcttatcggcatcacctgcgtcgccatgaatctgctgctctgctcctccggtgtgtactatatggacacgatcgcagacaccctgcagggcggcggcactattattatgaacggtgaaggggcagagagctttgatccgcagctcataacgcctgacgaggatctgaccatcgttgtcaatggagcacaggggcgttttcgtacgaccaactggtacatcacggctgtggtgacactgctcagcggcattctggcctattttgtcagcgggcgcgccctcaaacccctgcgcagcttcgcttctcaggtggagaaggtgcagctgaataatctggcggatatgagaaccaatgaggatgttctgccggagtttcggcagctgagtcactccttcaaccagatgctggagcggctgaacaacgcctttgccgctcaacggcagttcaccggcaacgccgcccacgagctacgcacgccgctggcgctgatgcaggcgcagctggatctgttttccgcggagcatcccgatgtgctgccggagacggcggaatttctctccctgctgcaggagcagacggagcggctggcgcagatgacaaaaacgctactggaaatgagcgaccttcaaacagtagcgcgtaccgaccaaatccagctgggaccgatgatcgaggagatcttcgcggatcttgcgccgctggcggaaaaaaacgatatcatgctggagcgaaagggcgacggcgccatgaccggcaacgacacgctgatctaccgaatgcttttcaacctgacggaaaacgccatcaagtacgaccgtcccggaggcgcagtgcgcatttccatatcccaggaggaaaagcgccttctcatccgcatcatggataccggttgcggcatcccgaaagaataccggcagagtatcttccagcccttcttccgggtagataagtcccgtagcagggaatacggcggcgcagggctggggctgtcgctagcatgggagattgccaatctccatggtggttccgtatgggtcgagaagagcacagaggaaggaaccaccattgctgtggaagtcccagcgtaataaatcaaaactccccattaaacaagtggtttgatctagccttataagagctaatcagctatggcagtttccttaaggagacatcgaatagcgcggtgaccacattttatcctttggcggcccctacccaagggcctctttgtttctatttcagattgatcgagctttcccagataatctgtcgccaactaaaacgtactgctctaaaaaggctttacacactggaagagcaagtaccgaaaacaaatcatccttatctttgaaataccgataaagggcacctgttgtaaggttagcaccggccatgatctggcgcaaggatactccggtaaaactatattctaagaattccttttggcacttttaagggtatcgccatgtgttttatcatattctgcaatcaatataacttcctccccgtaatgttgttatcttgatctttattgtcaagattttgagtatgaaatgtctcataatagtgcctaaaaatttccccacgcccttatctaaaaattacacatgcaaaagaaaatagccctttttaaatcgactctataatttgaattaacagcttgtcctcatcaaacaattcgtatagattattttggaggacaaataataaataatatagaaaaatttaatattgtattggaaaagctattgcaaaatatgtcgattattttcatttgcgtgacagtttaaataattataaagcgtttataaaatatatttagatagagcataggttgttccagaatttacaatagatctaaaaggatcgaacatgttgtagtaaaaggttattgaggaggcgatacaaatgtgtacagcaataacgtattatacaaaggatcactattttggaagaaatctggatctggaattttcttataatgaaacagtaacggttacaccaaaatattatccgtttcattttcgtaatggaaaagtgctcaatcatcattatgcaatgatagggatggcttatatagttgatgactttccgctttactacgatgcaacaaatgaaaagggtctcagtatggcaggactgaacttcccggataatgcggactataaagaagtgaaggaaggatacgataatattgctccctttgaatttattccatggatactcggtcaatgtgcaagtgtgagtgaagcaagaattctcttagaacagattaacttggtaaatttgaactttagtgaagagctgccgctttctccattacattggatgatttctgaccagcgagattccattgtagtagaatcaacaaaagatggtttgaaagttttcgaaaaccctgtaggagttctgacaaataatcctacctttgactatcagatgtttaatctcaataattatatgcatttatcgaaagaaccccctgcaaatacatttgctgccgaattggaacttgaacagtatagccggggtatgggggcgataggccttcccggagatttatcatccgcttcgagattcgtgaaagcagcgtttacaaagatgaactcggtttccggtgattcggaatcggaaagtatcagccagttttttcacattcttggctcggtagagcagcaacgaggctgcgtacatcttggtgaagataaatatgaaataacaatttattcttcctgctgtaacatggacaagggaatttattactatacaacttatgaaaacaaccagatcacagcagttgatatgtataaagaaaatctggacggaaacactataataagctatccgcttatgaaagaacagcagattaactatcggaattactaatacccttaaacataagttttgtaaataatctttgcatagcttttatattattcttttaggtgcgagatagtggtatatctaaaaattttctaatattttgaatttgaacaggctgcctcagaatgaaagtcggggcagcctatttgtgcttgaaataggagcattcctgcgttgcagtaatggcaaataacaagtgtagaataagcaggtactgaattaagagttaaggttatcttatggcacggattatgaagaacagaaaatgtaaaatagccgttgcgatgtttttcgttattctttttttggtgtaccactccttcacgcgggacatgattgcagcggcgaagactgcccgatttatcacttcatacaaatggcactctgacaaattatcggggctttaagtattgctacgacagtggagatattttttgttttctttataaacgaaatgttgaaactatgctttgagcatagagagatttcattcgtagatttgtggttctgccacataatcgacataaagccggtataggcctagccgggacttcgtccctgttttttcataaatcgacgcaatatatcgctgcaaggtgcgacgcgacatataaagggcatccgccatttcctgcacactctcttcggtagaaatcaaccgctcaaatacttcatgctctctctgcgtcagcgaaaaggattctgcaaatttttgagagtattctccccggcttttatttatggatttatccgccaatgtattctttatcacgttattcctgcggtttatatagacaaacattacaacgctgacagccataaacaaaaccagcgcagagataaccgttgcaaagcgatcatctgaaaccagcagcgcaatcgaaaaattagtaatcaaaacagcgctgatattatttgcggtacgccccataccggcccacagtgccggaatcctcatatagcgtgaaagctccatgaaactggcggtaaagaagacgacgaaaaaaccagaagacaagtagaatataaataatccgcccaagaatggaataccgaatttaggaaatacgacacacatgactgacatcaacataatgcagtacattatgataggcatatatttcctgtttttcaaatcaaacagaaaacctgccgtaagcccgcttgctgccagaagaaggcgcggccattgtccgatatccgtacctgccgcgtgttcaagcgtaaccgcgttatcgagcgtactaaaaatacatgccataagcgcaactaacagagcgagaaaaataccggtcgtaagcctgcctgttacccgtgccggagaaacaaccattttttcccgttcattctcttgcgaagcaacaggtttcctgcgcgcccgctctgccctcataaacagcaaggcaagaatactcaaaaaagcagaaagcacaatcgcctctgccaattccgcgttaattagattgttattgataaactgaatcagtattccaagcgcatacgatatccctaccaaacgggcaagacaattgttttcccctattgcacaggcggccatatcgtagaccttgccgctgaatataccaagcagcaagaataaaatgattccgaatatcaacgttgtaaagtaagagacgcactgctggatcacaaagatacatacgactgatgtcattactacgataaacaggaaaatgattcggtatgtttttttgatcaagcggtccagaaatggataaacgaaaaaaccggctgcgcttactcccaatatgtaattttgtgcgttaatagcctctgacggctttgccaaaagagaaaccatatcgacatacaaatattccgcgcccaaaaatacaaaagtaaaaatagccatcatcagtacggcggtcagcgacgctggttttcccagttccgtttttgtttcattccacatacttcgattccttgttaatatcatatctacatcatttattatacattgaaattcagttgattcctaccgtctgaaaacagtttggcgctgttgtgccacatacttttgatagtttggcgctcatgtggcctaccatctcatcatacgaaaagcaataataagggaaagcattttttaagatattcaaacgacaaaaccaatattttaggagggaaaaatgaaacagtgcgataatggtcatttctatgacgaagcaagatttgattcctgtccatattgtcaggaaggcgcaggagtagggaaaacggtagctgcgggcgctatcggaaaaacggtagccgcagtacccggatacggcacaggagaggctgatcgcggaaaaacggtagggatcatccagaaaaaaatcggcatcgatccggcggtcggctttctgatctgcatcaaaggcccgcatcgcggcgaagatttcaagctatgcgctgggagaaactttattggcagggcttctgctatggacgtgtcgctgacagatgacgacacggtttcccgtgaaagccatgcgcttgtgtcatacgacgcgaagcataaccgttttacgctttctcccggtcaggggcgtgggatcacctactgcaacgacgagcaggttgaagtagccaaacctctccatgcatacgatattatagaagttggaaaaagccgcctgctgttcctgccgctatgcggtgaaaatttccgttgggacgacgaagagcagaatgaggattgatcaatggaaaatataattgcatggctgaatacgcctctgacggaggacggctcttttcggctatggatgcttgtcgcggcatgcgctctcgccgttatcatccttttagctttcctaaacaggaagcacagacagaaaaaaacaaaaagaatagaacggaaaacggcttctgttacggagaagccaaaggtaaagcccaatcttgagattgctaatcttcaggggcttggaaaacgggaggagcaacaggacgctttcggtgcaagtctgttgaaaaattatgaggaaaacgggctgcttgcggtgctatgcgatggtatgggggggatggccgaaggcggcatgattgccgggtatgttgtgtctgagctattgcgtatattcccatggcaagattgtagcgaaccggaagagaaaatcaacaggataagttcccatgtttatcgtcagttccgcggacatggaggtacgacgctcgtcgcggcgttggtgaaaggtgggaccttgtctttctggtgcgtgggtgacagcgacctttttttgctgcgcgaagaaaagctctacgcactgaatatgagacaggaatataagaacgatcttttaatccgtgcattagaaggagctttcccgccagaagaggcatttatagatccacaggctgcggcgctttccgaatatattgggaaggaaaccatagtgtgtgaacataaccgcatgccgttgccgcttaggccggaagacacgctgctgctttgttcggacggcgtaagcgatacgctgacattgacgcaggttcgggaagcgatggctctttcgtccgaagaatgttgcaaaaagctggaaagggatattctttcggcagatatcccaaatcaagataattatacggtgattgccatcaggtatcacggaaaaataacggaggagtataaagatggaaacgaaaaagaaaatatcgactaaaaaaattatggcaatcgccttgttctgcgttttcgcgataagctgtgtattgtgcggaatatctgctgccagcagcatgggcatgacacctgctcaagcgcgtaatggcgtggcctatgtgcagcaggtattatatgacgtttccggtagccctgttgcggctggaagcggaacatgctgggctgtcggtaaaccgggagagcccgtggaatattttgtaacaaacgggcatgtggtgcagtatgcgtatatcgttcccaagcaagatccctcgtatagcgggaaggtaacggtagtttattccggtgccgagaatgattttgtagatgcgcaggttttatattattccggcccggaggaaaaggatatcgctattttgaaagttccaagcccgacagacaaacgcatcccgcttcccatcagaccgtctgatactgtgcagccgggagaaacagcttatgctctgggatttccgggtgtatcggatacactggcagagaatatccgctatgatatcgacgacgttaccataacagacggtgttatcagtaagcgcgcgtcggtttcgggaacgggctacgaagcgttccagatgaacgtagacatcaatccgggcaattccggtggacctctggtggacgctgacggcaatgtgattggtgtaaacacgtcggggctcgttactcagatcggtacggaggagcaatcggtaaatatcaacactagcgtaaactacgccagcgttgcggatcagcttatccgtattctggacgaggaacgtatcgaatacacgctgatgggtgaaaaaaactggatgttgtatacctttgtcgtaattggcggtgtaacgcttatcctcggaattgtatttctggttatggacagaaaaaaaacgtcggttctgtcagcggcggataccgagggaagttttgttgccggaaaaccggcaaaaaacagcccgtcaggcaaaaaaccgctgctacgcggcgtcactgggaaatatgccggacagagcttcgatctctccaaaggaaaggttacgcttggacgcgatccaaacctttgtaatattgtgttcgataagagtacgccggggatcagcgggaatcactgccaagtttcctatgatgcagccggggattattttctgttgatggataacggatcttcctacggaacgtttcttggaaatggaaagaaactgcctgcatccgtcgctgaaaagctggcaacgggagatacgttctatctgtgtaacaatgccaataaatttattgttgcaaaggagtagaaaatggcagcatattacttggaaaatgggaaaatacaggaggcatgcgctggatatgcctcccgcgaagacgcggaaatatatcatcttagtgccaacggagaaattacaacaaaagagattgtaccggatctgaaacctggcgaaggtctgctgatgtgtactgaaggtttttatgtggagtcgctggaagtacaagtagacttcctgaaagctgcggatgcggagcattggcttaaatatatggccctgcgccatatcgaacgagcgagatatattgatgacaggctttgggtgttggcagaaatgatggaggaaaaaatatgaatctggaaaaagtatgttacggctgtttccgggaaaaagagccgggagtctgcccatactgcggatatgacgatacagaggaacaaccgtttttagcgctgccgccggggacaattttaaacggacggtatatggcgggaaaggtgctgggagtaggcggtttcgggattacttatcttgggtacgacctgacgctggaaattaaggtagcaatcaaagaatatatgccgtcagggatggcgacgaggtataaagacggatatacggttacactcaccgggcgcgtggaaaaggaatatgcggcaggaatggaacgctttttggatgaagcacgtattctggccaaacttcaaaatttgcctaacatcgtatcggtacaaaattatttcaaggaaaataatactgcgtatttcgtaatggaatatatcgagggaatgagccttaaagaatatgttgcagagcatggaggcagtatttcctatactgaggcgcttgcaatcctgctccctgtcatggaggccctgtgcgaagttcactccctgaatctgatgcaccgggatattagcccggataatatctacattacagcatcaggagaaagcagattgcttgatttcggcgcggcacggttttccatgggtgacaacaaaagcgtatctgttatcttaaaacatggatatgcgccggaggagcaatattccagccacggaaatcaggggccgtggacggatatctacgcgatgggagctacgctttaccgatgtgtaactggaatagtgccgccggactcaatcgagcgcattcacaacgatacgatcaaaaagccctccgagttgggcatcagcttgcctacatcaatggaaaatgcaatattgaaggcactctccgtcaaagcagaggataggtatgctaatatgcgtgcgtttattgatgcgctgtccggtaaaaaagcggtatcggtaacggaacgcgtaacggcaggcgtaacgcaacgtgcctcgacgatagctcctgcggacggtagaagcgacttttgggattttatgaaaacaaatccgttgatacgttggatgattgtaggagctgccgcggctattttagtatttgcggtgattttccctgcggcgggagtatacaatgggaagaacacgcctataacctctaacggtggaacgaatgcccctgccgctacacaggaattggtcgtgccaagcacagagggcagcgccccggtgacaacaccggaaacggacgctccggctatggagatgacaacccatgatattactggttatggcgctgaaatctccgtcccggctgactggacggaagatccggaaagctgggctttcacgagcccggattcgcgtatggctcttggcgttgagctatacttctatcagccctatatggcttgttattccataaacgacgtcgagaacaatgtagaaacgatcgcagcgtgggcatcagaggaaatggggacaacaggatatgaaatcaaaacggcggggccgcaacaaataggagacgtgcctgcctaccagatcgacctccgcgcaacaaagcaaacaggcggagagattgacgtggtactcctttttgctgaaacgcaaaatggttttggattatatgatatcatgggagcttgtacggcagatgatgaagaagcgtacgcagcgcttcgcggatatatggatactttcatgattacaggccctgtcgatacgacgttcaggttgtattcaaaccaagagctgggcttcaaatttctgtatagcgcagattatatacaggaagaaccggctattgttaatgtgaaattcgatgggccggttatatcgtgcgtcgctctatatccttttgcaggagatgaaacacaatttgtagaggtggaaaatgtttctacaattgcggcgactgcacaagaagcgagtaatttcttttataacacccacataaacttgggagcggcgttgaacgagccatatatagatacatggggcggcgttgaatggacaatgtgggaaggaacattacaatcttcttccgttgcattcggtgcagcagagatcaatgggcagatatatgtcgttgccagcagggttcaggaatcaaatgtagagacagcaaatagtgtcagacgtgatgcaatgtcttccctgcgtccggtttgaccggacgcaagggacggaaaggagctatgatatggcagtggtcatcaaacaaacggtaaattgcccgcggcgtatggcggtttatgcgatttttgatacattagataaactaaatggtatttatgatcaggaacttgtgggagatatcaaagcgcaaataaacgtatttgataacttgagtgagtttgcttttgcggtgacggaacagggggatgcctctatcatacatatttccatactctaccctgcgccggaattgacggaggaaggacagcgacgcaccctcgtcttcttgcgggatagtattattcagcatattgagaatgaactcaacaccacagccagagaataaaaatcataaggcagatgtggttgtccgctgtttcggataaacaaacatggaggaaacgaaaatgaacggaaaagataagtgcaggattttaaaggaaatacggcaaaaaatagcagatgagaacgaaatcgaatatgtaacgagggattgtaaatttcagggtgaatgtagaggcacatgtccgcgttgtgaagcggaagtacgatatttggaagaacaacttgaacggcgtaaaaagttgggaaaacgtgtcgccatagccgcactggcgacaggactggtattgggcagtatcggctgtaccgaaagtgactctcggtttcaaagaggctgcgcgcccgtagaaagttatgatgatgaagaatggacgtcgcttgagggagaagttcctgcggacagcttgataaatgaacaaaacgaataaaaaaacggtttttccaacgattgctttggagcgtcatcggatgacaacagatggtattggtgttacgacgcttgttgcggcctacggctgtctactccgatgtcagtattgtctgaatccgcattcgcggcagcaagaaacgaatcaatgcgaatatacgccggaaaaactgttgaatgaggtgaagcaggataatctgtattttttggcaacaggcggcggtattacgtttgggggtggagaaccgttgctttacccggagtttatcaagatgttccgcacactcatgcctgccggatggaaactaaatatagagacttccctttatgccccggcagaagctgttattaccgcggcgcaggtagcggatagtatgattatagacataaaggacatggacaatagaatctacgaacgctataccgggcagaatgccgaagtaatgaagaggaatcttgccatacttcggaatacgatggatatgggaagcgtccgtatccgtgtccccctgattcctaaatataatacggaacacgatcaaaaaaatagcgcatatatacttcaaaagatggggttctccaacttagaatttttccggtatgtcataaagcaaccgggaaggctaaatgcagaataaatgaacataccgaatcaatgcagaatcaaatgattcaaagattactttacgtaggtttccgttttatctgtgatgaagtctgggctttatacagctcggacaacggcaggctgagtattggtattgagccggtggtgttggggaagtatttgctggtgggatacttgcatggcatagagtcgaagcggcgcatcgagcaggagatacaggtaaatatggcctatcgttgacttctggggctggattcagatgagcgggtgccggatcattcaacgatttcataaaacagatgcagcccgcttaatggaacaaatctgttttgtcgcctgcttgagcatatcttgcggcaatgcatagaaaaaggattggttgatggaaagatcactctgccccactccgcccatgcaaaagcggatgcgtcatttaaagtgaatgtcaaagtattggtggaacgtaaaaccatcgattacataaaacggttggatcgatacgaagaagcggagaatatcagaaatgtcggaagttatcaagccccagcgcgtaccgcacgggaaatggaaaccagcattggtgaagaaaacaatcaatacaatatgaccgacccggacgcgggaatgctgagacatccggggaaacctttggggatacattacctgcgtcaccaaagtgtggacgcggcacatgggatcgtggtggacgtggcggtgacggcaggaaatgtaaacgatttggaaccgtaccttgagcgtgtggaatatatgtgtaaccacatcggattaaatattcaggacacgggagctgacacgagttatggaactagcctgatctatcacgaaatgaagcgcatgggaatcaggctgcacacacccaaatcaacagacggtgagacatacaaggcagagctaaaacgtgaacattttcgatacgatgatgaagagaatgattactttgtttgcccataagccggatattgaaattgaagagtctggagcgagagtgctacaatatctgcaaggtctatcgggcgatccgcaaagattgttgagattgcgtgatactggagcaatgcgtaagcagtagccaacatagccggagcatccgggtaaatatctttgaagaagcggtgagtcagtaacggaagacagacgacacgcctgcccataaacgagttttagatttaagacagatatggtgcgagggaaattttgtggtgcaggagttgatacacaggttaaagtgcctgacaaggcgaggtaaggaagcggcagaagaccattgcctcctatccgctactgccttgaacatcaaacgcatgataaggtatctgggataactcctatgtcattattttttgctttgattttctaagtatcatcacttcgcctgagaaaaaagaaatagagaaaaaggccaatggctatgataaagatgtgggatttctacctgcggtacacagaagaatgtgtggaagtaccggacaggatcgtggaggcgatgtatgggcacaagcgtcaggaggaatccggcgaacggtatatctgccgttatcgcgcaaaaaagtgtatcaagctttaggggaggtctaaaagaatgtatttgcgctaatgatgtttgataagtatacaaattcaagctgtgaatcgggagaaagctaaagcatggtcaaaagaaaaaatacaaaaaagagaaaaaatcagcctcattaaggggtaaatagtccagaaaacaacaagacgtttaccaatattacaaatagaagattgaacgcaagtaaaatatttgtcatattgaagctcttgaaatttacgtttagacattgtattataaagaagtaaaaattgtttttagaagcggattatattccgcttttttgtaaaaagaattctgtgcggcaagaggcatcagcaggtaccattataattcattcacgctacaaaatttgctgtaaaaatagataacaagtatagattattagaaaaaagcattgcaaagctaagtggtttctttcatatgggggctaattagttggtaaaaaagaaaccaactttgcacaggtagacggttttttatttgtgaggtaaaggaggcctcatgggaaagaaaattcggcgctttttgtggagtagcttggtaggcatattaatcttatgtattgctatatttacttggataactttctatatggtcaatgaaaatgacaggacgattagtgatatagggaaaatttatatgtccgaaatgggcaagcaaatctcgttgcatttttccactgtaattgatctgtaccagtccaagctgaaaggcgttgtatggagcaatatgcgcaatgatataggcgcggcgaaactgcgagagaatttggctgccagtgcccaaagccttggattcagttatcttggcctttatgctgatgacggcagctacgaagctatttatgggaacccatacagatagacgaagaaagtgcctttatggatgcgctaagcgcagacgtgcaaaaggtaacagaaggcacgaaccagtcaggcgatgatcttcttttactgggaacggctgtttcttttcccatggaaaatggtgaaaatagcactgcgcttgttgcaggtatacccatacagactcttatagatatactctcgctcgatatcggtgaaacccgtgtttattctcatatcatccgcaatgacgggacatatgtaataaaaaatgccgatgcaacagaagaagattccgattcgtatttcgcccgtgtgctcaattacggtcatttcggcaatggtacccctgaggaagaagtacagaagatctcagaagcgatagaagcgggggagaaatattccatggttgcagagatcaaagatgaaatccgcaatacacattttaccccgctgggatattccgactggtatttggtatcagttcttccttatgaattgctgcatgaacctatatctcatctgcttgatcaacgtatttttactgccatcagtggctgtgtcatcattttatcggtaatgcttttaatatattataagtttttccgaatgtcccagcgacagataaagcttttacaagagacacggcaggaagcggagcgtgcaaatagagccaaaagtacatttttttcaagtatgagccatgatatgcgaacgccgatgaacgccattatgggaatgacagctatagcttcgacacatcttgacaaccggatacaattgcaggactgcttgaaaaaattgccctgtctagcaagcatctgctggggttgatcaatgatgtgttagatatgtcgaagattgagagcggcaagatgatgctgaatgtggatatactttctctgcgtgaagtgatggataatattacaaatatagtgcagtcccagatcaaggcaaagaaacagatattcgatatttttattaaaaacatacagactgaacatgtatactgcgacggcacgcgactgacccaggtgcttttaaacatactttccaatgcaatcaagtttacgccggagagaggaactattcatgtagcattgacacaagaggattcgccgttaggagaattctatgtgcgcaaccattttggggtgagagacactggaatcggtatgtcgcctgaatttcaaaagaatattttcgattctttcgcgcgtgaggataccaagcgcgtacagaaagtcgaaggaacgggtcttggcatggcgattaccaagcatattgtcgacgcgatgaaaggagcgatagaattaaaaagcgaagtaaataaaggcacggaattccacattattttggatatggaaaggaatacggaaaaagaagaagatatgcttctctcggcttggaatgtgctggtggtagacgatgacgagcagctttgccacagtgccgcttcttcgttaaaaaagattggcgtgaaggtggattatgccttagacggcgagactgccgttgaaatagcggcgacgcaccataaagagaaacagggttgccagattgtattactggactggaaaatgccgggaatggatgggattgtgactgcttacgattggaatgaaatcgaggaagaagcgcgcaaggctggagtcaacggtttcctttccaagccgctatttaaatctacacttttctacgggctcaggccttttataaagactaccctgctggaatcaaagccgctggagaaaaggattaatttcatcggtatgctcggcgacacaacggccacgggctttgtgcttgcggttatgatgtccaactcaggcagcgcgtgggataacgcgaagaaatatatcgagggcggtgcgcacggcggaaaaggcagtgaagcgcataaggccgccgttgtcggcgatacggtaggcgatcctttcaaggatacgcccggctcgtcccttaatattctgattaagctgatgtccatggtggcggtcgtttttacggcggttatcgtaaattacggtatactacaataaattcgaccttcagagtattaaatatattataaacaatatattcttaaaaaaatacatataaaatatagcacttttgcaatcttaaaccgcaaaggtgctttttgtatgtccttttatagggcacgagcacctccatttctccattttgatcgggcgttttcaaacaagcgacaaaatggaggttactatgaaaaaagtgaatctaagggagttttatccatctctctatacgaaagatacttatgtctttctaccggatgatgtagttactgctttatgggaagaaacaaaaagagaaagggcgggatatgcaaaaatacggtatcaccgcgcatactattctcttgaccgggaggatgggattgagcgatttgccctgcactcccctatgctgccggaagagatcatgcagcaaaaggaactgcgcgaatttctttattctatcattatggaattaccggaaaagcagctgaaaaggttctacgcctactatgtactgagaatgaaactgaaagatattgcgcggattgaaggaaccgatgccgctgctgtattacggtctgttcaaaagtcagaaaaaacgatccgcaaaaaaataaaaaattttttagaagattgagacaaaaaacggtgtgtttttctactgaataataagggagtatttttcttccgataaaaacgaaatatccaatcgtctgaatacgttagctgcatagcgagcaaaagaacgcacacgcgaggactgcctgcgggaatattcccgtcaataagataacatcaaaggcacgagcgggaatgtcaacgtccggaaacttccgtggctgggagtatgccatgacctatacagcctatcatgatacttgcgcgtagtcgagatcaagttccagagcgtgcccctgccgttggcagggtggtgagattccaatgtggcgctgcccgcgccggttcagacggttgcccgtccgttatgggaagtagtgtcgaatgataacggaatagaatatggaaagtgggggcagattttctgatctgaatatcagcacgaatagtctgccccaacttctgaatttatcaaacctctttgttgtaatttggaaatatgagttttttttgcatggagattgtttcggactataataagagcatccgccaaatctttgaaaggaggtgcctatttgtacgaaacaaagttgccatgtgagacctgcaaagaaaagtcaagccggaaatgaataaaaaatgaaaggtaaaaaatggaacatcaaataaaaccaccctgaaataagctggtaagccaagcaaaaagaatatgtgggctactgaaccgccaaactgcctagatgctccttaacccgtgcgtagtagatacgcaggaacttgttggctcctgccatcatgtagacgtaataatgcttaccctcgccgcgttttttgtcaagatattggaatacagcatcatgagagggcgcgtgtttgagcaggcagtccatgacctgaaaaagcgtctttctgagtgaggaagaacctcgtttggaaatgccggtactctgtgcttcaaaggcgccggactggaaaggcggtgcgtcgataccggcaaaagcaaccagcgactgcttacggttgaaacgtcgcacatcgccaatttcagccatgagttgaggtcctaacacattgccgaccccttgcatagccatgacaacaggaaattccggcaagccggaggcaagggaaagcatctgctgccgaatcagagccagcgtttccgatagggagttaagctgcgacacagcttgagtaataagctgtttggcaaaggtgcttcgaggcagtgtactgacttgtatgcaggcgaaatcgtagatggcagcggccttagtggaaagaaagttgtaacctgttcttttgcaccatttttgatagcgctgggtaaaaacgtttttggaaaggctgttgacgcattcaaaatgccaaaatttacccacgaagtcaatccatttttcgtgaccgtcccccttgcggggcgggctggagaacagcatgttgacactcggaaaggtttggtcaagcaaagcgatgaggctgtttttaagcataacactctgcttaacgtactggttgcactggcgggcgcaggttttaagcatgtggcgaacgtcttcttccggcgcatattgcggaagatcaagccaatggcttagagcatagctggcgattttaacagcatctatcttgtccgttttgacccgtctaagggaattttgaccgtagtcatgtacaagaatagcattgacaacggacacatagaggccggcttcgtgcagatgcctggcgacaggcagatagtaattgccagtatgctccataacaatgcgggtttcaccgtccaaacttttcagacgttcaaccaaacgtctgagttcatgagcggtgtgctgaatttcaaaaggtgaagcaaccacctcaccgaagggacgcaggatagcaaccatgcacttgcccttggaaatgtcgataccgacagcgttcataagtattcctcctgattgatgtattgtaatcggtgcccatctcttacccattgcctattcaatctactgagtgacacgaacgcacgagtggtggctctacctgcaaaacgaacgctgcaacaagaggatggctgactgtctcacgtacgggcgtgtagacccaagaaaggagtcgtcagaccaattactccccttattgtagcttagactatgggatggaaaggcgtatggctggctgccatatcctatccataaattattgtagtagagaaaggagagtgcatttatggaaaatctttcctctcgcgtctatacggtcaaagaagtagcaaaaatgttaaatatgaagccgaggaccgcttatgccttttgtgaatccacagataaatttcaagtagaacgtgtagggcaaagagggcttcgtatcaacaaagcatcatttgacgcatggatgcccagcggaacccaatcggctaatacgaaagaggtatagaaaatggcaatttcaataaaacaaagaggtaaaaaatatacgttcacattctattataaagacgaaaatggaataaacaggcaacaatatgaagcatatagcaacctggataaagccgatgaacgagcaaagatgattgaatttctgaaatggaagaatgatgataaaacgctgctacagttagtaaatgagtataatgcgaataaagcaggaacaaaaacaaagcattattctaaaaatgataatatgtgcaaaacattctcagagtttatttgggcatgggcacagcggcatgcgcataaagtacgaatgaagccaagttcgtacgcaggtttgaagcggaatattaggaatcacatcgagccatatttcggaaaaatgattgtgagcaagattacaccggaaacaatagaagattttttctttcaattaagccaaaagaaatgcaggggcgcaaagagttataaaaagagtgaagatcaaatacctactcttaaaggaagttcgctaatgaaagtatttaatattatccggcctgcttttcgggatgcggaaacatggggatatacgaagcgaaatccaataagcagtgatcaagccccggcatataagtatgcaaaacgaaaattctggaaaaaagaacaggtgcagcatgctttggaaaaaattaatgatcccgttttgcatttagctgtacatcttgcatttatgtgcaatatgcgaccgggcgaagttgtgggaacggatgctgaaggtattgatttggcaaataaatacttccaaatcagtcaagcgcttcagcgtgttgaaacagaagcccttgaagagcttgctcaagatgatattatccgtattttcccgaaaaagaaaccggacgcaaagactgtgatgatcctaaaaaagccaaagacagaaaaaagtgagcgcaaaggattcctaaacatgaaactgtgtgaggaaatcgagaaacgtttgcaacagatcgagcaagataagcgatattacggcaaggattatcatgactatggcttgctcctttgtttcccaaacggtgatccgattgaaccccggacaatggataagcgatttaagaagtggcaaaaaagtgatggggtgagtgcggaagatgtaattgatatgcaaggattacgaaaatctgcaacaatgtataaattgaggttaacaaactatgatgtgcaggttgtcggaggcgaaggcggacagacatcggctacaacgattcttgaccactatgacgaagttctcgaagaagatagaagaaagttatctatacaagtggaaaatgatttttatgggcggctgaaacaaaaacgggtaacagaggactttgacttgcgaaggttatttaaggagttagtcgaacagccggatttagcaaaaaaactttacgcttgtttacccgtgttgcagaaagcgacctgaattgcactcaaaatttatgagcaaaatttatgagcaaatgatttttgctcataaataatagatattggcagaacaaaaatagtagaaaaactgaagacctcgataaagatggtaatggaaaagcggtttcctacaaactcgtaaaaaaccgctctaccaaaggatttctttggagctgatggcgggactcgaacccgcgacctataccttaccaaggtattgcgctaccgcctgtgccacatcagcattatgaaatttttaggtgaaacgcaaatccttaccaaggatgtgctctacccctgagccacatcagcataataaaactgtgacttaaatattatatgatactccggcagatttttcaatccctttcaacggaagaaattttcgcttgcccctgggggtaaaaacatgtaccaaactattaaaaaagcataaatactttcacattttgtttttcttacgctataatgaaattattctgaattaattttatgaaaccctcccgtttcataagaaataaagggaaagaaggattttacaatgatttgtaacaactgtaagcaaagctacgacgacaatttgaacgcatgtccttattgcggcgcagccaaggcggttactgataacataccgccgcagcaatacggacaggtcccgccgcaggcataccaggctaattctccggcaaagggtacggcgacgggcagcctggtctgcggtatcatcgccatcgcgataggcgttttcgtcccgctcgcgggcctcattctcggcattattgcgcttaccctggggaataaggccaagtgcatgctcccggcggaccaaagaggtatggcaacggcgggctttatctgcggtatcatcggcatcgtaatcgcggtcatcttttggatcataaatgcagttgtggcggcttccatgttgtcttacttatactattgatcggagtgtaaaaatatcatgagaaataaacgcggaatttttgctttactcttactgttcatgatattgcttgcagccggatgcgcgtccagcaccgctccgacggttgaaataggcggcgaggtcctcccctccttatattccgtggtgggagaaaagaaaattaccggcacatcgaaaagtatcagcacgggacttgcggaggtagagcttacctatcagggcgtatcaatcgacgagctcaattcctatatcgagtctctgatttcggacggttacctggttacgcaggaagcgtcggcaacaggaagcggccagggctaccagattggaaaggaagcatccacagagggaaacatcattcttatcagcttttactttgaagacggcgggtctacggtcatcaattatgctgtaggcgcgggcaccattacgccggaaaccagaggctaacatttcccgctgaaaacagtctcccaaaaccgcaccgaggcgctgccgcggtgcggtttctatttcggcactgcgattatttttgtttggtccggcccttttttccgtataataaaagaaacaaatcctttgggaaggagcctccatgattttacattacgagaaagaacgcgtttatgcgaaagatgaaaacggaatgctgctggccgagatcacattcccggagacagcggacggatgggcggatatagaccatacctttgtcgatccttccctgcgtgggcagggcttagccgataaactcgtacgcgccgccctccagcagatcgcagaggccggaaaacggcccgtcgccacatgcccttatgcggtcaattggtttgaacagcatccggaggaattaaaagatttgttcggcccataaaaaggcttttaaatgggtgcttttgaacagcgcggccataaccaaacattttttttgaaaattttaaaaaatacttgcaggattttgaattcgggtgtagaatacatataataagaagatcatacaaggaatcagtaaaaaatggtttgaggaactgatttcagggtatgataatagtaaagacagatggacttcggcggatggtggtccggaagaacgtctgaatcgaaaaagaaagggcgtgataccaatgtacgattccgaatgcgtgacgttgggcacgcacgcacagtcccagaagtaggctttaaggtcgcacgaaagggatcacggaacaggatttttgaattggcagttgacggtttgaaaatatccgtgacagtggagcaaggttcccggagatgttgtgaagaaagcggagggaaaaaccggattccacggcagagttgtaaagaaagctcagtggaggcgccgaaaaagcaaacgtatcgcgggcgttgtagccgcaagggagtctggaacaattccagaccaaatgtgtgtggtgccgaaggtgtagcttgttcgcaagaaatgcggtaccggagcaaccggttggtacgtaaatacaaatactgcgtatcaatgtggcggtcggcagaaaccgatgggggatgcatgacccgaaggtataggcagagcgcaggcgcacaaaagtaaaaataaatgtaaatatggcaatggggtttccgaatggaaaccccattttttcgttttacgataccgcttcccgattcgcctcttcctcgttcttttcgcgcgaaatcctgatgtggagtttgcgctccagatcttttattttcccgtgctcacgcggcgtaatcagcgtatatgcttttccatccttgcccgcgcgtccggttcgcccgatacggtgtacgtaataatccggtttgtccggcacgtcataattgatgaccagatcgatcttatcgatatcgattccccgcgccgcgacatccgttgcgatcagcacccttgtttttcctttgcggaaggtattcatgatcgtatcccgttccttttgccgcatatcgccgtgcaggcaggccgacgcgagtcccctatggaaaagctctttttgcagctctttcaccttacgcttggtgttacaaaagacaagcgtaagccggggagcgcaccggccgatcagcccgcataccgcatttgatttccgtttggtctgcatataggcctgcgagaccgtttcgaccgggcggttctgtcccccgatcttaacacggaccgggtctttctggaactgccccgcaatcgccgtgatttccttgttcatcgttgccgagaacagcatggtctggcgctgctccggcacagcggacaaaatttctttcatatctccgagaaatccgtaatccagcatttcgtcggcttcgtccatcacgaccgtgcgcacatttttcagcttcagcaccttgcggttgataaggtctttcagacgcccgggcgtaccgacaacgatctgcgcgcctgtccgcagggctttgatctggattcccgcaggctgtccgccgtaaacgctcacaatccttacccctttcaggtgggccgaaagttcagccgcaaccttagcggtctgcatcgcaagctcgcgtgtcgggcacaggatcaatgcctgcaccttcctgttgggcggaaaaatattctccaggatcgggatcataaacgccgccgtcttccctgttcccgtttgcgcaaggccgatcagatcctttttttccaatagcgccggaagcgtctgctcctgaatcggcgtcggttttgtgtaccctatccggtaaagcgttttgttcatttcttttgataactgcatcgaaaaactcaaataactacctctttcccactccggcaaaaaataagactttgcctttcaaagcaaagtcttttcatcaatctactttgtgtacgtctgaagtatagcacactttcttccatttgtaaaatggaagaaagcttcagctgtccctccttaccatattctgcaaaacaggactgcttataacttattttgcatattggctcagatatcaaggaccactttctgaacccgatcttgattttgctcgatataccggaacgcatccgccatcctgtccaggccaaacttttgtgtaatcagtcttttcaggcatattttcccctgctttaccaggtcaatcgattccatataatcttcctctacatacatcaaagtccccaaaagcgtatattcacggtcctgcacatttgccagattgatatgcggcatcccagcaaaaacacctgcgaccacaatcgggatccctttcggcgagaggaaaagcgcttgattaagtgcggcttcatttgccgtgcattcatagaccgcgtctatcccatcttttccaaacactttttctatttcttcggcaagctcctgccgggatatattcacagtatgcccgatcccgcattgttttgcaagatcaagccggaaatccgagatgtcggtaatcattaccttcctggctcccattccttttacgctttgcgcaaccagattgccaatcgttcccgcgccgaggacaaggatattttttccttccacttcccgaaacgccctttttacagcatgtaccgcaaccgcaagcggttctatcaacgttccttcgtcaaaaccgacgttatccggcaggcggtaaaataaatcctcatccgcgacataatagtccgaagctccccccgggcattggcagccaagcacttccagcttttcacaaatattgtatctgcctgcccggcagggtttgcaggctccgcataccctctgcggccgtaaaacaacccggtcgccttttttcagctttgtattttcgcctgaaatttcttctataattccggtacactcatgtcctaacacaatcgggaagtccataaacggatgctctccgtaataggcatggatatcagagccgcatataccgatggctttgaccgcgattttagcctgtcccggacctatcgcaggctgttcgacttcgcggcattcaaaatttttaatcccggttaattctacctgtcgcatctttcgcctcccttaaaaatcaaccactactttaatagaatcctttttgccggcaaccgctttgtcgaaagcttcttgtgccttttcaaacggaaactgatgtgtcatgaccggaaggatatttgcccgcccataatggatcagtgtcatcgctttctcaaactggttcacataacgaatcactgttttataagtaaggccgcgcataaccgcactcgacatcggcataggggtcccgtcgtcgatcaaaaggcccagtaatgttatcgtcgccccgtcccgcacatatcctgatatatcatagaatgtcttctcggttccaaccgactcaaacgcatatcgcgccccataaccatccgttaactcccggattttttccgcaacatccccatccctgggattgatggtatctgtcgctcccattttcttggccatttcaagcttaaacggctccatgtcgactgcaataatggttccggcgccaattgttttaagcgcatgtatggtcatcattccaatggttccgcagccgacaacgaccgcgctgtccgcgtatccgatcccgctgttggtcacgccctgcagcccgacggtgaacggttcgattaacgcaccttcctgataggacatatcctccggcatttcatataccaaaaattcgggccacgctacatactcgcacatgcatccatcccaaggcggcgtacccataaaatacatattatggcaaaaattataccggcccgcgcggcattcgtcgcagcgcatacacggttttcccggttccacaatcacccggtcgcccacggacaggcggctgcatccttccccggccttgacaacctcacctgcgcattcatgcccgagaatcaacggttttccgttcatggcataatcgccgatttttccatccgtataaaaatgcaaatccgagccgcatatccccatggatttaatgcgcaccaatacttctccctcttttacgtcgggcatcggcaaagcccgtatttccatcttccgcggctctgtcagcacccatgctctcattgtttccattgatatccacctcattatttaaagtttgtttttccgcgcttccttatcactcctgtcaggccgccatttcatttttggccaatttccctctccgcacattatccagcaggagtgccagaagaataatcgctccctttgcaacatcgcgcaggaatggatttacgttctggagagtcatccagtttgagatgacctcgataatcaatgcccctgcaaccgcgccaataatatagccgttgccccccgaaaggctcgtcccgccgataacaaccgccgcgattgcgtccagctcaaggccttctccgagggttgcggacgcagacataagtttggagctcaaaataacagaactgattgccgaagtaatccccgcaatcacgtaggcaacaattgtagtctttgcaatactgattccggagtaccacgcccccttcgcattgctgccaacagccagaatgcgcctgccaatcgtaaaccgcttcatcaggaggattgctactacggttaccgccgcaaatatccagatcggcgtcggaacctcccccagcttgcccaagccgaagaaatcaaagccttccgccacaattgggaattggcgtcccgatgtgatgtagagtgcaattccatacgtaaccagctgcatcgccagcgtgaccataaagggcggaaaattcaactttgaaatcatcaggccgttgcaggctccaatcgcaatccccgttgctacggcaatcaatatgacgacaggaatagataggcccgcggaaaagcataacgcgctgataattcctataatcgtaacttgtccgccgacagaaaggtcaatacctcccgtagcgataacaaaggtcattccaatcgccagaattccggtagtagctgtccgctgcaaaacgctgaccatattcgttggagaggcgaaaagcggcgttactatcgtgactacgaggcacagtacaaccaatatcaaaataattgaaaactcggatgccaatatcttttttactttttctctcgtcatttgtttgtcctaccttacatatagatttgcatttttgctttgtctatttctcttgccatgaacgtccccgcaatctttccctctttcagtatgattattttatccgacatgttgagaacctcttctatttctgacgacataacgacgactcccactccttgttccacgagggcattcatcagttcgtataccgcaactttggcgcctacatctatgcctcgcgtaggctcgtcgaatacgacgatctttgattgggccgctatccactttgcgagtacaaccttttgctggttcccccccgaaaggctactgaccggatattcgaccccggcgcacttaatttgcagggctgcaaccatttcatccataatgccttttacttttttccggttaatccatcccagtctggaaacatcctttagggacgcgaggattatattatctaaaatgctcatttccgtaacgagcccctcttccgcccggttttccggaaccagccctatttttctggcaattgcctccgacggctgccgggcggtaatttttttgctatcaaggtaaatatctcctgccacgcggggatgccccttgccaaaaacgccgaacaacgccttggctgtttcggtctttccggcccccaaaagtcctgcgatgcccaggatttctccccggtgtaccgaaaatgaaatgtcctccagcagcccttctacggagatatgctcaaaacgcagtaattcttcccccctggggaatacctttttcggatatttattcttcagcttccgccctgcgataagttctgccagtttttcttcgtccagttccgccgacccgtattgcccgattttctgcccattccgaaatacgatgatctcatccgtcacttcgaggacttcttggagcttatgggaaatatatataacgatatatccgaggtcttttagccgcttgacagcacgaataacggcttttccgtctttatccgtaagcgcagacgtcggttcatccaaaataaccaccttgcagttctgtgagagcgcacgcacgatcgcgaccagctgctgatgggcaaccttcaggtctcccaggcgcgtatgtgtgtcgatatcgatttccatcatgtgcagtaattctttcgcttgtttatgaatttttttccaattgatatagcctgctttgctgcccgttaaatgagagataaagatattttccgcgacgcttaaatcggggagcatattgagctcctgatatacaatccctacccccaaatgctgtgcgtccagcggggatgaaatttttaccggtgttccatctgcaagaatctttcctttatcggcaatgtaggctccgttgataatcttcattgtggtagactttcccgcaccgttttcgccggctaagccataaaccattccgctgtgcagccggaaactgatatcatccagagctttaatacccccaaagcttttacagatcccttttagctccaggctttcctgtatcatctatattcaccactttctcccgatatccgtcttgtttccctgttcccatcagggcggcgatatacgcaccgccgccccgcttgcaaaattgcttcaattcataaagctattccagatatcttccgtaccagaccacagctctgtctccgtttttacatcatacagcgcccacagggtcgggtcgcttgtatccgcgcctgtaatgacccgggtttccatagggatcacttcgccgtccagtgtctctcctttagaaacgatctcaagacatcctttcgccgctactgtcgccagcgcaagcggactctgttccacgcacacatccatcaaaccggaattcagggcgtctacgccgctgggatcacaatcgattccagaccagtagatatgattctcctcgccgcctttcccggtttttccgttttggcgcagggcggaaatcacgccggggtccatagagtcacagtgcgtaataacaccgaacagatccggattcgccgttaaaacgtcatttaacgacttttccgccgtatcgcttgcccagtcgcatggactttcaatcagctgcattcccgtttcggccgctacctcgtcgattccatcctgccggagataggcgtcactctgcgtcatcgttccctgcatgacggctaccttcggattttcaacgcccaattcttttgctttatcagccagccactgcgccgcactcgcacctgtggccacattatcgctcgatacgaccgcaaaattgaggttgtcgcctgaaatttctttattaaaaccgatgcactgtattcccgcatttaccgctttttgtactgccggagccagcgcttcgctgtctgctgcatggatcgcgataatgtcacagcccatattgataaaatcatcgatttggctggattgttcgtttgcatttccatcgcagttgactaacgtaacttccgcacctgcggtctccattaatttcacaaaatactcggctgcgcttacaatataggtggacgataggtcgctgaccgttaatccgacttttagtccatcgcctttgcccgccagctctgcggcaaaaccattgcctgccgccgcgccgtccccttcggaaacctgggcagattcttctgccggggctgccgcgctttgttcagcggtttcgaccggctccgcagatgtctgcgctgccggagctgcacacgcggcaagcattgctgccgccagtaaaagtgccaccacaaccattgataattttttcatgttctcctcctgatatattggattattttcttttgccccaatgaggcaaacttaatttttttcgatagattccggacattcctgctttttcaaagcccgccgtaccgagatacgccggtctccgatcaactatgcggtcacataggtgtgaaattctagccattagaaaaaggcacaaaaaaaggcgccttttccagcgccgataaataaaaatacaaaaaaaacgattggttaaaaaactacacttttttcaccaacgttccgtatattctgatttcataaagctttgatacagggtagtataaatagccgatatcctaaacaggatcgttttaaagttaatcccctttgcttgtactttaacacagtccaatatacatgtcaatattcttttagcgcgtccattctcctcctgcgctggcctgctgcccacaaaattgcataatctgcgcctttttgccattttttccgctttttggatcttccggtaaaattttatgccctgaggttttgtcttcaaaggtatcttctgtgggcaagggtttgacaaagatgattatctataatataatcctgtgtgtagtagaagccaatcgaaaacattcctgtatctttgcatgtaaaggataaatttttatcctgcagcaaatctttatttgtttttcatcttttttcgatagagaccggattttgccgggcttttgttttatcatgctttcttttgaggattcatgccgggggcgcggtaatacgcatgcattttatacagaacatacatattacaaaaggagattctaatttattatgattagcaaaccatattcaacagatttcaggctcgacggaaaaattgcactgatcacaggtgccgcttcgggcatcggtctcgctatcgcccagctcttttcggaacagggcgctactgtatgtcttctcgatcggaatataaaaagcgcgcttggagcttcggccaacatccccggttcttatgcttacggtgtggatattgccgattcggcatccatcgaagaggcgatcagccaaattctaaaagcccacgggagaatcgacattctcgtaaacagcgcggggatcggtacggtcgaatgggcgaaggatttcccggaagaagattggcgcagcgtaatcgatataaacctgaccgggaccttcctgatatctcagcgggtaggccgtgaaatgattgccatgcaggagggcggaaaaattatttgcctcgcttctcaggcaggaattgttgccatcgacaagcatgtcgcttacagtgccagcaaggcaggcatcatctctatggtgaaatcccttggctatgaatggggaaaatatggcattcaggtgaatgcgatctctcccactgctacggaaacgccaatcatcgtcggatattgggatgtcggcaaggttcatgaagatgcgatcgccaatactcccgccgggcgcttttgcaagcccatggaagttgcgctggcagccctgttcctggcctgcggcgcttccaatatgattacgggctccaatctcgtaatcgacggcggttataccattcattaacggtaccgttcctcctcccaggcgtgttctgtgccgtctgtccggaatacgcctgggatagaatatccaaacctattgcatttatcttcttacaatccgctgtccaatagtatgcgcagtgtcaggaggtctctatgacaaaaatacccgaataccggaaaatatattccgaactgaaaagggaaatcaagcgtggcacctatagcccagggatgtttctgcccaccgaaacggagttggaaaacatgttcggcgtaagcagaactaccatacgaaaagcaatcagccttttggtactcgaaggattcatttccgtacagcaggggcgcggaacggaagttcaggaagtctccacatcgcaaaggctgaaccagatcacttccttttcggaaaccttgtctcaaaagggctatatcgtaactacgcgcggattttacctcgaacatattcccgcgcctgcgtttgtccgcgaagcgcttggattggagaaagattgcacggttcatcatttgcaaagagtgcaatgtgccgatgggcgcccgatttgtattatggagaattatatcagtgcccatataatccccgatttcgagattcgcaacagcaattttgtcagcctgtacgagcttttggaacatgaatataatctcgttctgcgtgaggctgttgaacgtattaccgccataggcgcctccttcacagaatctcaaatacttcttgttccttcaggcaccccactcttattcagcaagcgtatcacctactgtgataaaggaccttttgaatatgtaattaacaaagtgcttgcagagcagtatgaatatgcaattcatctttcgggaagggcttaggacctaattttccagcttggtcccagaaaaatatgattcgataaaaaaaccgccccagccaaatggctggggcggtttttacctataaatgattgatttattttccttccgcgaggttcttgtagtattcgtaccgttccttcgcttcctcttcggattttgcaaacagcttgtccgccatttccgggaagagtttcttcaaggatttatagcgggtctcgctcatgatgaaatcctggaagcttgccgttgccggtttggaatcgagcgtgaacggattcttaccctcttccttgagcgccgggttgtaacggtacagctgccagtagcctgcttccaccgcgcgcttttcttcgtgttgtgatttgcccatgttgataccgtggttaatgcacggagcatacgcgatgatgagggacggacccggataggcctccgcttcctgcatcgccttcaaaagctggccctggttcgcgcccattgcaacgcttgcaacatagacatagccataggtcatagcgatcgcgccaaggtctttcttcttgaccttctttccggatgctgcaaacttcgcgatggaaccggtaggcgtcgccttacttgcctggccgcccgtgttggaataaacttccgtatcgagcacgagcacgttcacgtcttcgccggaagcgagcacgtggtcgaggccgccgtagccgatatcatatgcccagccgtcgccgccgaagatccagacggacttcttaatgaacaggtctttctggtccaatatcttcttgcaggtatcgcactccgccgcaaccttcccaagggccgcctcgaggttcgcagaagcggcctttgactcgtcgcccttgtctgctgcttcaagccatgctttcattgcttccacaacttccgcgtccttctcaccgggcgcgtcgatcgcagcctgcacctgctctttgagggcgttcctgcgggccgtgaaggcaaggttcataccatagccgaactccgcgttgtcttcaaacagcgagtttgcccaagccgggcctttgcccgcgtcgtttaccgtataggggcacgtcggagcgctgccgccgtagatggacgagcagcctgtcgcgttcgcaatcgtcatcctgtcgccaaagagctgggtaacgagttttacatacggcgtttcgccgcagcctgcacatgcgcccgagaactcgaacagcggctttaggaactggctttccggaaccgtattctttttgatctcgatcttcggttcgggcagcgccgctgcaaagtcccagttctctttctggagtttttcctgctctgcaaggggcttcataataagggccttttcctttgcggggcaaatatccgcgcagttgccgcagcccgtacagtcgagcgtagaaacctgcatacgatagttgtagccggccttgccgcgtgcgggcttcgtcgcatagttcgccggcgcgttcttcatgtcttcgtctgtcgcgaggaacgggcggattgccgcgtgcgggcatacatacgagcactggttacacataatgcagttatcaatctgccactccggaaccttgaccgcaatgccgcgcttctcgaatttcgtcgttcccgtcggaacgaagccgcgcggatcgaaggcggaaaccggaagctcgtcgcccttctgcacaaggatcggatggatcacgtcgcagtaatatttgtcgtcgggaagcgtcaggcagggagcgccctgcgtcgtggccgcccagctttccggatagtttacttcctcaacagccatgcctgcgtcgaccgctttgtagttcatgtttacaatctcgtcgcccttcttgccgtacgttttcttgattgcctgcttcatgtactcgatggcgtcagcctccgggatgatgcccgcgatcttgaagaatgcagactgcataaccatgttggtcctgccgccgaggccgatctcgcccgcgatcttgattgcgtcgatattataaaatttcagtttcttcttggcgattacgttcttcatgaccgccggaagctccgtttccatctcttcgagggaccagggggagttgaggaggaacgtgccgccttccttgattccttcgagcacgtcataacggatgacgtaggacggattgtggcatgcaaccatatcgggatgcgtaatgaggtatgccgactggatcggggatttaccgaaacgcaggtgcgaaatcgtgatgccgcccgacttcttggagtcgtaggagaagtaaccctgcgcatacatatccgtatggtcgccgatgatcttgatagagttcttgtttgcgcctaccgtaccgtcggaaccgaggccgtagaatttcgcgctaaagaggccgtgcggcgaagaatcgatcatgtctttcacttcgagggacgttcccgtcacatcgtctgtgataccgaccgtgaagtggttcttcggcgtatcctgcttcatattgtcataaaccgctttcaccatggaaggcgtatattctttggagccaaggccatagcggcccgcataaaccttgatacccgcccggcctgcttcaaagagcgccgttacgacgtcttcatacagcggttcgccaagagaaccgggttctttggtcctgtcgaggacggtcactttttcagccgaagccggaatcgcatccacaaacgcgcttgcatcccacggcctatacaggcggactttaatgacaccgagtttttcgccctgcgcgttgaggtagttgacggcttcttccgttacgtcgcagccgctgcccatgataacgacaacgtgcttcgcatccggtgcgccgacataatcaaacaggtgatactggcggccgaacactttcgcaaattcgttcatcgtttcctgaacgattgccggcgtcgccacgtaatacttgtttgcagcttccctgttctggaagtagatatccgggttctgcgccgtaccctgctggtgcggatgatccgggttcatgccacgtgcgcggaactcctcgatcgctttccagtcaaccatctcggccagtttgtcatagtcgaggagctcgattttggaaacttcgtgggacgtcctgaagccatcgaagaagtgcacgaacggaaccttcgctttcagcgtggaaagatgggccaccgcagccatatccatcgtttcctgtacggaagcggcagccagcatggcaaaaccggtctggcgcgcagccattacgtcggcatggtcgccgaagatggaaagcgcgtgtgccgcaagcgcccttgcggaaacgtgaaacaccgcaggaaggagttccccggagattttatacatattcggaatcatcagcagcaggccctgggacgccgtaaacgtggacgtaagagcgcccgcagcgagcgaaccgtggacagcgccggcagcgccgccttcggactgcagctcggaaattttcatcgtctgtccgaagatattctttcttcctgccgcggcccattcgtcgcaggactccgccatcggcgaggaaggagtgatcgggtaaatcgcgccgacgtcggaaaatgcataggcgacgtgcgcggcagcggtattaccgtcgattgtttgttttgccattcttagtgacctcctaattttataattcatttaaaaacattcgcaacattataattatagtattacgggcactaaaaagtcaaggcagagcgccgctatatcccctttttttgtaattttggcagcatgctccgggggcgtataaattcatccgtatgtacgtacattttttattttagagaaagaggcgttttcttttccaaaaccatgccttgtactccatcctttcctgtgctatacttaaggccacaacaaaaaatgtgcagagtagattttgcgcgtcaagtgtatcaggatgggatgtcgcctgataacgaaaaggcccttgccttgcggtgcaaagtcgcgtccgctgctcacaaaagaagattctttgaagcggcttttgcttttttgcattttggccgacagcctttcttttgtagaagcgttgccatttttacgaaagggaggttatttttatgtccaaaatcagtcccaaaaccctgcgcctcgtgtattgcgcaacctttatcgccattgccgttgtagtcggcagttttctgtctttttacctgacggaaagtattaaattcaaccttgcgcccgtagttatcatgctgaccggcgcggtgctcggccccatttggggcgcggcggccggcggcgtgaccgacctgctgtccttcctcatcggcacggccgcaaaacccggtccttattttcccggctttacggtgacgatgatcctttacggcctgatatccggcctcatcttttaccggaaaaagcgcccgtccgagataccgtcgattgcaaaaatttccctcggcacggcgcttacgcagacggtttgttcgctgctcatcaattccttctggaattacctgctgtacgggccgacctacctcgtggtgctcactacgcgcctgccctccacatacattatgtgcgcagtgtatatcgtcctgatgtgcatcttgctgaaaaacaaacaaaagatgttcaaatccctttacgtgcccgttgcggcgtaagcaggaaaaaagcggcacatccgccgctttttttgtttccttttttggcagaggatttcgaattaaaacgtgaaaagccggttcctgagaaccggcttttcaaaaaataataaaagggtggggattgacatatcctagtctcctaagatacagtctcattttatactacatccggcaggattgcaagtgataatttgttaataatttatgaaccctgccttttcacttttcccgcgctttcccaagcctcctgagcacataattcggcagcgcgaagcagccccggtgaagctccgtattgtaataatccgtatggaggccaagcgcgttccacgccgccgcatcgaacacaagcggatcgcggtcctgggacgcgaacccgaacagccagtggccggacgcgtaggtgggcatatggaactgatagacccggcacacgggaaatacggaggaaagttttttatgcgcgcgctccatctcgaccgcgtcgccttcataatagggactttcgtgctggttgaccattacgccgcctggcgcgagcagcctcgcgcagtcttcataaaacgcctgcgaaaaaagcccttcccccacgccgaccgggtccgtggaatcgatcaggatcaggtcgtatttttcctgcgcctcccgcacaaaggcaatcccgtcgcagaagtgaagagaaacgcgcgggtccccgagcttcgacgcagtctgcggaaggtattcgcggcacaggtccaccaccatccggtcgatctccaccatatcgatatggcggacgcccggatagcgtacaagctcgcgcaccgcgcccccgtcgcccccaccaatgataagcacgttttttgcatctgcgttcaccgccatcggcaggtgcaccagcatttcatggtaaatgaattcatcccgctcggtcagcatgatgaaaccgtcgagcgtaaaaaaacgtccgtattcgtaggaatcgtaaaaatcgatcttttggaactcacttctcgtatcgatgaaatgatcctttattttaatgccaaatttcgcatttcccgtaaaatattcataaaaccagtcatttttcaaaatttctgccataaaaaatctccttcatctcccgctccaggttccgctcgatgcgcgcgcgcgtcttctccttcaggtccgccgcgtcgagattgaacaaataattgtcaagatcatatttcttcaaaaccatgctcgtgtggaacacgcgttcctcatacaggttgacgtcgtatgtgtcatatttttcgaggatatgcctggggataaaatcctggatggacataatatcgtgatccatgaacaccttgcctccgttttccgtgcgggtgaatccacgtacgcggtagtccatagtaataatatccgaatcaaagcttgtgattagcttctcgagcgttttcagcggcgatatttccccgcaagtggaaacgtcgatatccgcgcgaaaggtgcaaaccccgttctgcggatggctttccggataagtatgcaccgtcaggtggcttttatcaagatgtcccaccaggctcgcgggcacctcttcctccgcaatcagcatcgtgacagacgcgccctgcggttcgtaatcctgttccgcgatgttcagaacctgtgcgccgatgcggcgcgccacgtctgtcaggatctccgtcagacggcgcgcgttatagcattcgtcgatatattcgatataactttgccggtcctcttttgtgttggcataacaaatatcgtataaattgaagctcaatgtttttgtgagattattgaatccgtataatttcagtttttgcaaaccattcctccgcaccagaactgttttatttatagtttcattatatatcaacgaacgggaaatgggaaccatttatcccggcatggggatcacacttttgtcactctttcgtcgtgcttccttatgcaggacgtatatttgcctttcccggtcatctattataaatagtaccggataagaatgtattcgcagcccaaggaatacctgataaatcaagattggtctgccaatacagctaaataaggaggaacaacatgaagtttcaactcgcaacagattacgcaatacgcatcctgtgctacctctatgaaaacaacaacaggctttccaccgcgacccacctgtccgaaaagcttgggatcacatacctgtatttcatgaagctgacgggcgtattgaagcatgccggactgatccagtctgtccagggctgcaacggcggctaccagctcgccaaaaatgcggaggacgcgacgctttatgatgtggtgaaggtgatcgagggcggtattaagatcaaccgctgcctcgaggaagaccgtttttgcagcagggacgcggcggaatggtgcaccgtgcacacctttttccaggaacttcaggacggtttcatcgagcggcttgacagcgtccgcatccgcgacctgtgccaaaaaccggaaaagcagactgccgcccgtgaatacgcggccctcgaggtttaacggcaggcatccattataacgacaggaggaacattgtacctatgaaaaaaatacggcgactaaccacggctttgctcgtgattattttcctgttctccataaccgcgacggcgatggcggacggtgcgcccagtcttgttgatttaccagttacaggcttattgaacacagaatatacggaaacaacagatacggaagatacggaaacaacaacagatgcggaagaagacatgggtgccgggtctgaagcgcccggtgcggcagaggaatccacgacggagggcgcgtccgcaccggacggtgataatccttcgccttccccttctccctccgtcccggaggacggcacggcggcggaagccccggtgggaatttcgcttatgtcgcttattcccggcgcggacgttacggcaacaacctgggaggacctaaaggactccgtggagcaggcagaggtcgacggaaaaataatcgctctcgacccggcccttgcggggaccatgtccgccacggcagaactggtgatcggccacaataacagcgtggtaatcgacggcggcggcctcacgcttggcgcgccgtccggcggagcgcatttccgcattacaaattcgggcacgggtaccgttaccctgaaaaacatgacgcttgacggcaccggcggcacaggcagcgtcgtcctttcaggcggcggcgcgaagctcgataccgtaacggtcagcagcgtttccggtacggctgtctccgccaccggcacagacagcttaacgcttacaaacgtaagcgttgcaaacgcggccgcaggagttgcggcaagcgcaggcgcgcttaccatttccgattcctccttccaaacgatctcaggcacggccgtaacggcatccggcacggctacgcttgatactgtgacggtagacggagcaaaaaacggcgcggctggcgggagcggcctgctgaccatcgacggttcggaattcaggacggtcgccaccgccgccattacgcttggcagcggcggcgcggaggttacggataccatcattgacggtgtgacgaacggctccggcgtcgtgacgggggcgaatacactcaagcttacgggttctgcgatcacgaatgttacaggtacgggcatcgctggaaacagcggcaatattaccgtagacggctgcacattttcggaaaccaacggtcacggcatcagcgaaggaaaagacgtcaccgtcaaaaacacattgtttgaaaatgtgcgcaaccagcgcggcggccatggcagcgcaatctatgccggcacgaacctcacggtagaagcttcaagctttgtgaacagcgcctccacgctggacagcggctatattcagggagcgatcgtcggctacggaggcagcgggaaaacgatcaacgtaacgcgctcgtacttcaaggacaacaaggcctcccgctacggcggcgcgatcggcctttaccagtacggcggcactgtgaacgtcagctacagctattttgaaggcaacggcgtttccggcaaaagcgcaaacagcgacggcggtgcgatcggcgtctacaacaacagcagcagcgtactttgtacggtgaacgtggataacaatacgtttatcggcaatactgcgggcgacgacggcagcgcgctctttttcgagggccgcaacgacatggtggctgcaaacgtaacccataacacgttctatggcaataaatccaccaaatatttgctggcggccgcggacagcggcggcgtggtgcagctttccctcgatgtggtcggtacttttaccaataacacgttcatcggcaacactgctcccaattatgcaagcaagcatggggccggggcggcggtcggcgagcatatcgactccgcgaacgcggcggtgcgtcccacggccaccttcaaaaacaacattttcgtgggcaacggcggaaacggcggcaatagctacgcctcccgcaatatcgacgtcacggacggcaccgaccttggcggcaacgtaggctacgacaacggcacggctgttgcggcgaatatcacggcggagagcgtattcggcacttccccgcagccgcgcgcgaacaacacgcatcacggcgcggcgggaaaagcgggcagcgggtatacgggtatcctcacgaccgtcgtcatccaaccgaacgacggggtaacgggacaggcggataacacagccggcgcgcccgcttacggcacggatgcaagaggattcacgcgcggcgcctccaattccgatgccggcgcgctggagatcaaattcgtgaaattcgacgccaacggcggcgcgtggagcggactgcccggccttacctacgacggctccaaatattatgcggacgatacggcttccacgggttacttcctcgtaacggacccgggcggcagcgtgagcgtactcagcggcgaccttcccaccaatggtccgcttgtctttgacggatggtatacacaggcagacggcgggacaaaggccaccggcgatgtggccgcggccgaccagacgctgtatgcgcactggaaatccgcagcggcggaatacaccgtgacatacgtgggcaacggcgcagatgccggtacggtccctgccccggacaccgtgacggagaatacgctttaccaggtaaacgccaccccgcccacgcgcaccggctttacgttcggcggctggaaggcggacgatgcttcgggcacggtctaccagcccggcggctcgttcattatgccttcaagcgacgtaaccctgaccgccgtgtgggcgcccgttccggtcacatataccataacctatcacggcaacggaagcgacggcggcacggtccctgccccgggcacctataacagcggccagacagctgctatttccggccccggaacgatgtcccggacggaccacagcttcctcggctggaacaccgatccggctgggaacggtacgggatatacggaaggccaaggattcctgatctcaggaaaccttgacctgtacgctcaatggcaggataacgggcggccggccgtactctataccctgacttttgattcgcagggcggtacatacgtcggcccggtcacaaacatcgctgcgggaagcaaggttgcagcccccgcgccgcctgcacgcacagaatatacgtttgatgggtggcaccatactgcggactgtacatgcgcaagcgacgatccgtgctgggattttgaccgcgacacgataaatggccataaaacgctgtacgcccggtggatcccggcggcacaaacactatatacggtgacgtttgacgcacagggcggcagcggcgtcgccccggttacgggaatcgtacccggttcacggatcgcggagccagccgcgcccacgcgggacggctatgtgttccgcggttggtatcaggagagcgaatactccagcccgtgggtatttacggagcacacggtgaatggcaacctgacgctgtacgcaaaatgggaagcatcacctggcgccggtacggatgccggcgccgcggataccccaaacggcggcggtaaagtggaaagcaccgctaaaacaggcgatgcctccgccccattggcggtactgattcttgccgcggcggcggcagctgcggtgatcttccgcgcggtatcgacgctaaaaaaacgcaacagttaacagcctctgccctgttcctctccgggaacggcgcggaaaagccccggacagtgtgcccggggcttttcgtatatgtttcacattactaatccccctgccgtgcagcatccgccagggggattttttccgtttcaccggcagcgccttccgctccggacggtttggatgacagtaaaaaacggatgcgcttctagcacatccgttttagaatcccagtcagttattccccggccggtgccgaagactccgaaccgctttccgccgcttccgccgctgtcggcgcgtggccgaagcggtactcaatatccttgccgcggatctcggcgatctgcatcatctgcgtaaccgtcacaaatttatagccttcatccttcagcgccttgatgatcctgtcgtacgcatccacggttgtggcatggatatcgtgggacagaacgatagcgccgtcctgcacatatccgccatccggggtgccgttgaccacatggtcgtacacggtatccgggtcgcggttttccttcttccagtcgttcgggtccaccgaccacaaaatctgctcgcggccaatctgctccgccatgtcctcagacatagagccatacggcggacggtcgatcagcgcacgcaggcccgtcgccgcttcgatcgcatcgttggccttcccatactggttcgtcatgatttcatcaagcgaaagcttcatcaggtctttatgatcccagctgtgcgtgccgatctcgtgtccttcgtcatacacgcgcttcacaatatccggatactcggctgcgttggtcccgaccatgaaaaacgtcgcgaccgcatcgttttccttcaggatatcaagtagcttcggcgtgttttcgggatgcggaccgtcgtcgaaagtaagcgccactactttgtcatttaacggatcgatcccgtcaaggctcttcggggccatgtatccttcctttgcctgcagctgggcgaggctagtggttacctcgggcgtgggctcgggcgtcggttccggcgttgccgttggttcgggcgtcgccgccgcggacggttccccggtgggggtcgtggtaatcaccgtgggcgcggcggaagattccgccacgctgcccgtgccgccgcatcctgccgcaaacgcggaggccaccagcaccgcaagtatcatagagatcaatttcatttttttattcattcgttattcctttcagcggtcttgggggaaccgccgcttcaattataatacacatactgatatgttgcaaacaccagcggccagcgtgtatcaataaattcccggtatgcggctctttccgtcattcctccccaacagcttcacccgcagctggagcgctcctgaacaaatatgcgggcgtttctcctctgagctccgcgatctgcatcatttgcgagaccgtgacgaatttataacccttttccttgagcgcgggaataatacgcgcatacgcgtccaccgtggactggtaaatttcgtgggacaggatcacaacgccgtcctgcaccacgccgccgttccatccgttcattacatgctcatagatggcatccgcatccttatacttccaatcctccgggtccaccgaccaaaggacctgctcgcggccaatctcttccgcctgctcctccgtcaggttgccgcccggcgggcggtcgaaaagggtacgcaggcccgtcgccgcttcgatcgcgtcgttggccttcgtgtattgctccaactgctccgctgtggacaggcccttccattccgacgcttccggatgggtatagctgtgcgtagcgatctcgtgtccttcctcatattcccgcttcacaacgtctggatactcctcggcgaggttccccaccacaaaaaacgtcgcgactgcgccgttctccttcaggatgtccagcagctccggcgttttgaccggattcggcccatcgtcaaaagtgagggccaccaccttgtcgttcatcggatcgatcccgtcaaggctcttgggaagcataaagccctccttcgcctgcaattgctcaaggtccgttacttgcccgggagtgggctcgggcgttgccgccggttcgtcttcttcgggcatatgggatgcggcggcagtttgcccgctcgtaatcactgttggctctgcggcggccgccgcatcccccgcgccgcagcctgcaagcagagccatgcaggcaaggacggacagggtaatacagaccgttttcctcatcattttttatcctttcagcagtctctgaataccgttctttagattatagtgtacttgtaacaaagttgcaaactccttttccccggtaccggcgtatacaaaaagataaccgcagtatactgcggttatccggtcattttatcctgctgctttgcatcattcctcttcgccctgtccggcggaatcagccgcgggcgcactatagaacttaaagccgcccatatcctggccgcgggcttcggcaatctgcatcatctgggtgatcgtgacaaacttgtagccccggctcttgagttccttgatgatacggtcatacgcgtttacggtcgtctcatggatgtcatgcgacaggatgacgccgccgtcggaaaggtagccctccacttcctttgctccgccgccgtccccgccgttcatcacgttggaataaatgatatctggatcgcggtaatcggtcacccagtctttcgggtccatggaccagatgatctgctcccggccgatggacgcggcttcctcctttgtgatcgctccgcccggcggacggtcgattagggtgcgcaggcccgtcgccgcttcgatcgcgtcattggccctcgtgtattggtccaatttctctcctaccgataaattgggccattctttcgtatggttccagctgtgcgtgccgatctcatgtccttcgtcgtagacacgctttacgatatccggatatttctccgcattctgccccagcatgaagaacgtcgcaaccgcatcgttttcctttaggatatccagaagcttcggggtaagcgtctcgtgcgggccgtcgtcaaaggtcagggcgatcaccttgtcgcccatcggatcgatcccctcgatactttttgcggtcatgaagccgtcccgctgccggatctggtagatatccgtttcggctggcccggccggggccgtttcctgcgcagttccggctgcggctgcctgctccgccccgaggaccgcttccttgttcccggcattcagtatgcccgcaagccttgcaagcgggactcccacctcaaagcttcccgccccggaaggcgcgatcgtcccgtcgccgaagaaaaacagcactttatccggcgctaacacgaaattcgcataattggcttcctcgggagccgttccctgtgtgaacaggctttcatccatatttttcagcagtacttcattcctgcgcagatattcctgcgcagcctgcgcaacctgcgtgaggtaatcctgtgacggatcgaacacatccgaaagcgcgagctttttgcctgccgcggggtcgtacacaaacgcatcgacttcctccgccgcagcctgccccgccagctccgattccgtcgtaaactttatactgagcaggttcccttccgtaacatacggcttataggtcatcgtcaggctgcacagcccatctttgttttccccgtgcgcagcgtccgcagacgcgcggaattctgcgagcttattttccgcaaatgctttcagctctgccgagatatccggcgcgttcgcgaccaccggataatcgacggataccagggtatctccttccgtttccaaaatatgtccgctcgttatcccttccgccgaatcaagctgcctgctcaccgccgccgcttcaaaccgtccccggtaggcttccatgtccccggttccatttcccgcgcaacccgccgcaagcggaagcgccaacgctgccgccgcaaaaagcgcgatccatttccgtttcatactttttcccccgcgccggacgcccaatacccggcctttgttcctatgcttgccgctcccagacctgatccgcggttttgaagcgtctttcgccaccaaaattattttcccatattataccacagaacctatatttatcacaatttgtttccgcatgccgcgtgtaaccttccacgacggagtttgtaatccctttcccaatatgatacgatactaggtacgagcaggcgggtgcgttatggattactcaaaaaagagcctttgggcttttttgccaaacaggaaaagcgaaacgaaaccagtggatgtcttttacgtatatcccactatttacgcgcacccattccagaaaaaacgccatcatatgagcatgaggaatccgatctacctgtgggtcgccaaggggatgtctgcctggcagggccagctttttgcgcgccattgcaatttttacgcgccgcattaccggcagcttggcacagaaagcttcaaaatgcccctgcctgaagtcatgcgcgcggaacggatgccttatgaagacgtacgcgatgcattctactattaccttgagcattataacaacggacggccgttcatccttgccggacacagccaggggagcgccatgctgctccagctcatgcgccgggaattttccgatccgcggctgcagaaaaagctcgtcgccgcctatttgatcggcttctcgcttacccggcgcgatttcaagcgttatccgcatctccgccttgccggggcggcggacgatacgggggtcattatttcttataacacgaccgcgcacggccttcccctgatgcggtttatccgcccggattcgctttgtgtcaacccgctgaactggcggcacgacagtgtatatgcggataaatccaagaacgacggcgcggtgctgttccaattcgggaaaaggttcaaatacgaggtgccccactatacgggcgcgtatgtggatgaggcgcgcggcgtgctgatgatcgacgacgatgcggcttacgagctttacaaggcgcggtggttcttcaaaaaatttctgatgaaccgtggatcgctgcacatgctcgatatcgcgcttttctataaaaacctcgagcgaaatgtgggggaacgaatcgccgcatatttgtcccggccttccgaatgacggcgctgcgcgcccccgcaggataaatccgcagtaaaaaaaccacggatactcaatccgtggtttttagctctttcggctttgtgatgatgcccgcgaacagttccgcctcgccattttcgtcccgcgatacccggccccggcaatggatccacacccattttccgtccttatcgcgcacccggtattccaaatcatgcgtatcggtggccccgtcgcgtatttcctccatcgattgtgcaaaggcagggcgttcgtcctcatggatcagcatgctccatatggaatctccgccatacacaacctctcccggaagcgcaaattcttccaccattttcggcggaaaacggaacatattcgtcttcatattgcagatatagatataatcgtccgtactggccgaaagcgcctcgtagaggtgctccttatcgtaggaaaaattccccggcatgcccttttccgcccgctcacgtcccatcctgccgttgtggtatatccgcttctgccggtacatccgttcgtccacttccgtggtgatcttggttatatcttccatgtcctgcgggccgacttccagcactccatagcaaaagctgatctcatacggctttttttcccgttcccggatccttgccagttcctcgagcgcatgctgcatgaccctatccgccacccgttctccgcagccgtaaaacacgaccataaattcgtccccgctcatacggaaggcgaactggcctttttccagcgaacccgtaaccaccttcgcaatcgtggtgagcaaattatctccctctacatgtccgtaggtatcgtttaccgttttcaacaggttcacatcatagaggcacaccgtaaccgccgcgctttcttttttggcccgcgcaagcacttccgaaagccgctccttgcctgcgcggcggcccatcatccctgtgagctcgtcgaggctggcctcccgcgacatcttttttgcgctcgtaatatccacggattgctggaaatgcacgatgcgcccgtccagccagcgcatcgtgctgtcataattttcataatgcctgtgcgtgagcgtattgtattcctcccacaggtaggatggcttttccgccggattgttccgcagctggtcgatcgggcagaaatcacaacgctgcgtcttatccgcctgcaaaatcttccagcatattttaccgataggttcctccacgccaaactctttgcgcatggtcttattcataaaaagaatttcgtccgtatcgagatccgttacatagatattcgcccgcatattatccatcaactcgttaaacacccacgtctgctccatctggttctggcaatagatccggttggcaagggcgatcctcgaggtctgcgcgagcatttccaacagccttttttcctcttccgtccattcctgttctttttccgccatgattacgccctggatgcggctggaataagaaacgggaaccaccaacaggggcgcgtcttcttccgtccggcagtccaatttcatgatcctgtcaagcttctcatcgtctgcggcctcgtccgtccgggcaaaatccttccattcactgaaatccagatcaaaaaaatgacggaccgcctcctccggcaggatccttccattgcgccacaccgcggcttcacggacccggtagtcttcggagaggccaatgagccccacgccgcagacaggcaaaaaacgccggataaaaacggcaaagctttcgatgatttccgcaagcgggccctgcccgatcacaaagggttccagttcttcgagcgcttcattcaggatgtttaaatattctgttttcccacagttgccgctcattaaaaaatacccttccacgctagtatgttttaaagatattgtgtttattatacgccttcgctatatgaaaaacaatcatatttcttattttaacaaaatccatcccgcccgctgaaacttccgctttttatcactgcttgggcgttccgtccagtcatttttaattgtaattgtttttcaattacattattgtacattataacgcttcctcaaataaattacaatattaattacaggagaagcagcggtatggaaaaattcaaggtcaatacaaacgacggcaaaatttcgtccatcaaccggacgatccgtttgaagccggaatattttgaaaaaattatggagttgagtgaaaagaccggcgtttccttcaacaaaatcgtgaaccagtgtattgagtatgccttaaataatatggaagaaaaataatgcagatatcaaaaaagacgttgccggagcagcgtcttttttgatgtttccatttactgaagaatgccgtactgtacgataaccgccgcaaaaacgaccgccaccatagacatcagcttaatcaggatattgagggacggaccggacgtatccttgaaaggatcgcctaccgtatcgccgacaacagcggccttgtgggcttcactgccttttccgccgtgcgcaccgccctcgatgtatttcttcgcattatcccatgcgccgccggagttggacatcataaccgcaagcacaaagcccgtagcggtcgcgccgccgagcataccgactacgccgttcgcgccgaggataaggcccacgatgatcggggcaacgaatccgaggatcgccggagcgagcatcaggtgcagcgcgcccttcgtgcagatgtccacgcacgattcgtaatcaggctctccttcgcctgtcatgattcccttaatctccctgaactgccgccgcacttcgacaacgatcttcatcgccgccttcccgaccgcgctcattgtcatggacgagaacaagaacggaagcatcgcgccgatcagcaggcccatcaggaccgtcgggtcgagcagggagagcgccgacatatcgatctggcactggtccgcaaacgctgcgatcaacgcaagcgccgtaagcgccgcactgccgatggcaaagcccttgcccgttgcagccgtcgtatttccaagcgaatcgagcgcatccgtacgttcacgtaccaccggatcctgaccgctcatttccgcgaggccgcccgcattatctgcaaccgggccgtaagcgtccgtcgcaagcgtgatgccgagcgtggaaagcatgcctaccgcagagatcgcaacgccgtaaagaccgacttcaaagctgccgctgccaagcgttccgcccgaagcaaaatagctgatgagcacgctcgcaaccactacgatgaccggaaccgccgtggatttcatgccaagagcaatcccgctgataattgtggtcgccgggcccgttaccgtagactccgcaaggtctttggtgggcttgaagtggtcggacgtgacgtattccgtatagtagccgatgataatgccggcaacaagaccggaaaggatggccacatacacgccgacatggtccggcccgaggattcccgttaccaggaaataacccgctacggcaacgatcgccgctgcaatatacacgcccttatgaagcgcggaaagcaggttcttctgcgaagcgttctcctttgttttcacaaaaaagctgccgatcacgctggcaacgatgccaagcgccgcgagaaccatcggaagcgccagtccgccgccgccgaggcccgccgcaaccgcgagggcgcccgccgaaataatggacccgacgtaggattcgtaaaggtccgcgcccattcccgcaacgtcgccgacattatcgccgacattatccgcaatggttgccgggttgcgcggatcgtcttccgggatgcccgcctccaccttgccgacaaggtctgcgcctacgtcagccgctttggtgaagataccgccgcccacacgcgcgaacagcgccatgcacgaagcgcccatgccgaacatcagcatgttgctcgcgatctgcgccgtatcgcccgcaaaatacgcgtttagtataaaataccagatcgtgagatacagaaggccgaggcctacgaccgtcatccccataaccgcgcccgaagagaacgaaacgcgcagcgccgaattgaggctcttcgtcgcgcccgtgaccgtacgggaattcgccgccgtggcgattttcataccgatgaaacccgcgagcgcggagaatacgccgcccacgatgaatgcgatcggtacgaagaaggtcatgaagcctgttgcggccaagatcgccaggacgatggttacgatgacgaaaaagatcgcaaccgtcttatactggcgtttcaggtaggcgttcgcgccccgcctgatggcaccggcaattttcttgatcttttcgctgccttcgctttttttcagcacaccggatgcagcgaccgctgcgaacacaagtgcaatgacagcgccgatcaaggcccaaaacataatgtccattggtacttcctccttatgattgcatatatttgtagaaactcttatacaggcgcgcccgcaccgcccaaaccggatatggcaaaagcgcgtcatctatttcaaatatggaaatcggccttccgcgtcctgccggagcaaggccgcctttgcttgcttcttcttgttgctgaaaagttctacccgctgcccgcgcggcttttccgccgggtttgcacggagtcccgggctgtctgtcttgatgaaaacccgtaccgggagcggcaccgtaaaagtagttcgaaaacctgaccagcttcattataatactttttttgtttatttgaaagtaaaattggcaatttattcccgctttttttgaacaatttcaatgaaattctcaattttttcgaacattgctgaaaaatatgcacgatttcccattttgacgggatttgacaggtggatttggataaattataattgaattgtactaatacacttaatacagagataggagacgctgccgcgctatgatggtaaagcttgacccggcatccaaaaagccgatctatgaacaaatcgtccaggaggtaaagtcgcttgtcatgacgggaaagctgctgccgcatgagcaggtgctttctgtgcgcaaggcggcaaaggagctgggcgtcaatcccaatacggtccaaaaatcatacgcgatcctcgagcgggaaggcatcctttactctgtgacgggaaagggcgattttgtggcggacaacgccgcccgcatcaaggagatgaaaaagcaggaaatccgtgatatgttcatacaggtcacgcgggaggcgcgcgattccggtttgtggatcgatgaaatattcaccatcgtggacgaggcctactcgacaaactgagaacgggttttccgctcttgcgccgttccgcacgatcagacgtccacagccgcccgaagggcggccttttttatccccggccccggaaacccacgttcccggcggccttattttaattttcccggcggttttggagtcttgcggaaagcgtataaaataattatcaaacggaaaggacaaacagaaaatgctcgatgcggttcgccgtacaacatgcggaaaaatatgcgggacggtggaaaaggacgtccatgtatggcggggcattccttatgcgcagccgcccataggtccgctgcggtttcgccccgcgcagcctgtctccgcatgggacggggtttatatggcaacggcattcggacccgcctgcccccagcgcaaaagacgcgtcgggacgagcgaggactgtctctacctcaacatctggtctccccggccggacggtaagaagcgcgcggtgcttttctttatccacggcggttcgttcgcgggcggggcgggcagcgatcccgaatacgacgggacgtccctggccaaaagcggggacgtagtggtcgtgacggtcaattaccggctgggcgtgctcggttttctcgatttctctttcctaggggaagatttctcgccgaactgcgggctttccgatatcgttgccgcgctcgcatgggtgcacgggaatatcgaagcattcggcggagacccggaaaatatcacggtgttcggccagtctgccggggcgatcgccgcctccgtactgcccgtaatgccttctgcgcggaactatgtatctaaagttatcatgatgagcggcggaccgtcgcttttgtatacgaaggagcattaccgggaaaccgcacggaaattcctttcatttatgaatatctccacgccggaggaactgcgcctgatccccgcggagaagctggcggcaaaacagaaaaaatttgcttcctgctgcggcctcggcgacggaacctttatgatcgaggtagacggagcgctggttcccgattacccgattcccgcggcggcgcagggcgccgcgagggatatccctatcctgatcggcacgacccgggaggagctttccttttcctgcaaaaagcttctttccagggtgctcgatatcggaagcatcttaaaatcagaccgcaacagagaaagcgcagagacccggcagcggatcagggaggcctacagacggtatggacgccgtgcggaagccatgatgctgacagaccgtgttttccgtatggcaagcgtatggtatgccgaggtctacagccaatatgcgcgcacatggatgtaccgtttcgattatgaaaccccggccatgcagcttaccgccctgcatgcctgccattcttcggatatcccgtacgtcttcggcaatctccatgcccggcagtataaatggatgttccttctgcccgcgccgcgttcacgccgcaaagtgctcgcggagattcagggggatttcatccgctttgccaaaaccgggcttctcccgtggccgcggtgcggcagcggtatgaccccggcaaagtgctatgacaaacgctgccgcatcctgcccatggtggagccggagatcaagcgcgaatatgaaaaaagcgaattcaagcgccacagctttaaagggcttgactatacgggagccggtcagcgataatagagggaaacaagctgaagatcggaggatgccgtatgacagatctatcggaagtccggaagctccttgcggaatattctacgtgcgagataagcgaaattacgccggaaaagcgtttaacaagcgacctggagcttgattccttttccctgcttgacgccgttgccgcctgtgaagaccacttccgcctttctatcccggacgaggatttaaggcgcctcgataccgtccaggatgtggtggactatatcaacgcgaaagcaaaatagcgaaaagagcctcaaaagccgtattgcgtctcatgcgcaggtacaatctttcctgggcaggtttcgccgcccaaggccattctgtcagcggcagcaacattttaaaacttatacaaataagtttagccgtgatttcagggctgacaaccctaaccagaaacggacgacggacatcatctgcatacatacgaaagaggtttgatccgctttcccctattttttctttctcgagaggttccagatggaaagcgcgtaaaacgcagccgccgtaattaccatgaccgcaatacatgccgcgggcgtcgtcatttccccgccgaattcaaatttcacgccaagcgccgtatcgaagtcccgcaccatgctttcgggcgcgccggcaaaggaaaccgcggcaggttgctctgtcatcactgtgcggaaaaaagacgcggagtaagagaccggaaacgcccggatgatcccctgcaccgcctcgggcagactgccgatgggaatatagacgccggtaagaaagccgatcagcgtgccgatgacagtgctcgccgttccgaacgcattctggcttttgaaaaacgagacgataaaaagcacgatggagctcgacgacaggaccgaaagaaaaatcccgccgatcaccttgagcatattctccatggaaagcacctccccgccggacgcaacgataaaaatctcgccggcaaccagcgcaagcaggctcatgatgacgcccacggcaaacgcgcagaaaatataaccgcccgcgaggctgccccgtccgatgggggacaccgtaaaatccttgacgatctttttcgcgcggtcctccaccatgatgccgaacgcgcccagcgtggacgtcatggagatcactgcgaggatccccgcgatgatccagctgttcatcagaaagtcgatcccttccacatcttccatgccgcctgtaatcgtgtcgccgaggaacaccgcatacagcgcgatgatgataaatacggcgagcagggaaaaaaacaccgagcttctgtccctgaagaatacttttaagttgcgttttgtcattgcccacataatcagttcctcacttccgcgcctgtaatgttcaggaaaacgtcgtccatcgttccccgccgtacctcgaatccggcaatctcttcccggcatttatcgataatgccgattgcctccgctgtgtgccgcagccggatgataaaatctccgcctgttttttggaaagcgatcccttcccgcttcaggaggccggaaagcttctcttcccgtttgggcgtgatcttaagcatatcccgggtataattttccttgagctccgcgggcgttcccttggcaagaatgcgtccgcggtccatgatggtgatgtagtccgcctgcgccgcctcttccatgtagtgcgtggtaaggaagattgtcatgccgcgctccctttgcagcaggcggatcgtatcccataccttgcggcgggtctgcggatcaagacccgttgtcggttcgtcaaggaatagtatttgcggcgtattaacaagagcgcgggcgatatccgcacgccgccgctgcccgccggaaagctttccgtacgggcggttccaaaaccccatcacatccgctgtaaacgccgcggatgtgaccgcgtccctgagtgcgtcttttcccattccatagaggcttccccgcagcagcaggttttcgcgcacggtaagcagtgcgtcaagaacgctgtcctggaaaacgatgccgatttccgcccggatggccccgtcttcccggcctagctcgcggtcgtccaccaggacccgccccgcatccggcgcgagctgcgtagatattatgtcgatcgtcgtcgattttcccgccccattcggccctaaaaacgcaaacagcgctcctttttccacataaaagtcgattccattgacagcccgtacatttccataggattttttcaggccttccaccgtgataatttttgtcatgcttctcccgtcctttcggtttttacagggtttacgttatcaataaaaaaagaccgcttcaagcggttttgcgcaaggtgcattttttctatgctaaagtgcagaaaagccgcccggctacagggacaggtggaacaggcaggacaccgggaaaacaaggataagcgcgggcagcatattaacagccttgacgtccttgattttggcgatggcaaagccaagcgcaagtgtcatcagcccgccgacggcaataaaatcggccaacatcggttcgcttataaggggcatgataaaccggctggcgtaaaagcaggcggtaaggatcaaaaactgcgggaggacaatgataaggatcgcagagccgagcgccgtggcaaagataagggacgcgaaaatatccatcgcggccttggaaagaagcaccgtgaaatccccggtcatcccctcggtgaaagcgccgaagatattggtgccgctggcgcagaagaccgtcgccacaaccacgtaaaaattcatgtactccttccggtccccttcgatcttaaaatgcatgcgggagatcgctttcccaaacagggcgcggacccggccgtccagccgcagtaattcccccgccaacgttcctaggataagcgacaggatcacggccggaagggaagacagctttgtcagggagatcaccccgatggcaatcgcgcaaatcccgaaaacagtattaaggggctgcgaaatgcgctggggaaccttgtcctttattttagccccggcgagcccgcccgcgacgatacacaggcaatcgattattacccctaccggcatgaatgtttcctccctcgtatggtttcaaagacggtgtaatataacataccgggctttggaagtcaagcggaagtacaaataaaaaggcgggcttccgcccgccggaccggcagctccggtcatttccgtttcatttttttgatctgcttattgatatcctccgcgtccgctttgtttttgataacaagcacaccaaaggtcgcgaggtatacgacgccgatcatcccgagaacaattggcacgtagggcatttccatgggaataaagcccgtgggcccgccgatcaggaacaccaccgcgacaatatcggccaggtcgacaatcatctgcagcgccgggctgctgatcggcagcctgtcggtaaaagaaatcatcaccgcgatacacgtcgtcatcaggaacaggaccagcaccgcttccggcaccacggccgcaaaccccaccgtaaccgagagtatcgtaaacaaaagcatcagtacggtaaaggaaacgcaattcatggtaacgtaaaacttaaatttcgacatcttccttttcctccttacaggccaagcttttgcttgagcgtttctacataatggcgtgtgacgatgactttttcgccattctcaagctccgcctccatttttccgttcagcagcgcccgcacatttttgagcgtcattacgttcaggatgcacgatttgctgatgcgcacaaaattagcctttgcgacctggctttccagctcgtataatttcaggccgcattcatagacctcttgttccgtataaacgaaggtgcggttatccaccgactcaaaatagaatacatccccgagccgtatctggaaggtctttccgtcccgtttggctatgacggaaaaggaatacagcctgatctgctcgatcagtttttcaagtccgggatcgataagcccgcatttgatggtgacctccacctcttcattgtccggcgactggtcgatcagaagtttcaacccattccctcctcgttacggcctgtacggcgcaccgtcccgcattcgcctgcggggcatgcgtcccttttgctgctccttgcgcggccttccgtcaattggtaaaaaatccaagctgcctgcccgccggttttttgcgcgtatgcgcggggccttcggcaagaagtccggaaggaatatccgcaagaaaaggcgagcgttcttcttgccttgtgagcataacaagctcgtcctgtgcgcgggtcatgcccacataaaacagcctgcgttcctctccttcgctgcattccccatccttcctgcggaagggaatcaggccgtccgttacgccgcacaggaatacggccgggaattcgaggcctttggccgcgtgcagtgtcatcagcgtgaccgcgtccgcggtatatgccttctgcccgctgcgctttaggtcgccttccgttccgagcgtcagggcggttagaaagtctgccatgcggtgatggaacaccgccatgttcctcaggcgtttcaggcacgcgggcgcttcttccccatatccttgccctgaaatccatagatcgagaagctccgcaggagcagccttgcgcatcagcggcgcgcaggtttcaaaatgtccggcaagctttgttccccccgcatcctccaaaacagatacaagcgaagctgccgtttgcttcctccgtccgtaagcgtccaatattttttccgccactgccggggcgacgctgtccgcccgcaggcaggtcccgagggaaacgctgtccttcgggtcgcacaggatgcggaaaaacgcgagcgcgccgcgcacgcggcggtcagtgagcgtattatcctttcccagcaccacataggggattccctcttttacgaggcattcctcgatcagctccgcctgccggtgcgtgcggtaaagcacggcaatatcggacaggccataagcggtgtccgcgctttttttatgctgcgcatgggcggcaagcatgtcgaccccgcccaccatagcgttaatttccttcgcaataaacagcgcctccgagaagggagagtccgccgctaaaagccgcgtttttacaccgctttcccgctgcgcttccagcacaggttcactgcggcggagcaccgggagggcgcagccgatgatttcgggcgtagaacggtagttctttttcaggcgtatttcacgtacaggccggtcctctttgaggcgctcaaagcaatgcgcgtccgaaccgcggaagccgtaaatagattggtccgggtcgccgatcacaaaaattcctttgctctttttcccccatgcgcggatcaattcgagctgtacgggattgatatcctgaaattcgtccacaagcaaatgctcaaagcgcggacagagcgtttcgcactttgcgccgccagcacggaatttctccagcgtatcggccaggatatcgtcgaagtcgagcacgccgagcgagcgcagccgagcgcagtaagcgtcgtacaccacctggggaatatcgcccgccgcgccgttcttgattttagaaaccgcctgtattgcgtcgcggggtttcatgacacagttacacgcggtaagcgtttcggaaagaaccgcctgcgcttcctgtccgtcgatcaccgttatatttttatcccattctttcagcaggctgagcccaagggagtggaacgtgccgatgtgcattgcccgcaccgcctttttatcgccgaattgcgtctccagcctctcccgcatttcgcttgcggctttattcgtaaaggtgacggccgtgatcgcttccggcgctacgccgcactgctcgacaagccatgcgatgcggtacacaagcgtacgtgttttgcccgtacccggccccgccagcacggcgaccgtgcgttccggggcagatgcggctgcccattgttcttcattgaggccgtaagggtttccgcccgtttccacgggtgccgcctcttttgggctttcgtccgccttaggcggtgccgcctgcgcggacgcatgtttttccggtttctttttgggttcgttcgcaagcagggaaagctggccggacagcgcctgcacctcgcttttatccatcacgagaatctttccgtattcgccgtcgtagcccggatggatttccacctcgccgcagcgcaggcggcggattccctccgcgatgcacacgcctgccgcccgttcgatttccgcgagcggcgttttgcgcaggatggtaagctccggaccgagcgtcccgataagctccagatattgcgcgcgcaccttcttgctcgcaggcgtaagccccatcgacgaagctaccacctcgggcagcggcacgatgctttcaaaatgctttgcattttccggccgaaatccttccgcgcggtccgcaagctccaccacacggtggtagacgcccacggtgatgcgccgcccgcagaccgggcatttgccgcccgcggcggccgtctcctccggcgtcatgcacaccttgcagttccggtgtccgtcgttatggtatttcccttcctccgggaaaaactcgagcgtcccgtaaaattcatccgtatcatggttttcgagcgccgccgcaatggcgggatagctcatttccgtattgaagagattggcttcccgcgcaaggttcgcgggagaatgcgcatccgaattggataccatcgtgaatccgtcgagcgcagacagccgccagttcataggcggatcggacgacaggcccgtttcgagcgcatggatatgcggcgtcaggtctctaaagcattcttcgacggcgtcaaagcccgaataggctccgaacagcgaaaaatgtggcgtccaaatatgcgccgggataaagactgcctccggacagatatcaagcgtgatctcaagcaggtcccggctcggaaggccgaggatgggccgtccgtccgaatgcaggttgaacgagagctcgagcttccccgccagcgcctctgccgcctcgagcgagggcagcaggatcacattgtggattttgcgtaccttgccgtcctgtttatagatagagctgatctcccccgaaaggataaaccgcggcgatgcgggattgcctcccacctcatccgcaaggcggtattcctcttttaagcggtacaggccttcttcggcaggagccagcttttgcttcagttcctcccgccatgcgggatgcgtaaagtcacccgttcccagaaggtcgattcccttacggcgcgcccacaggtcgagatgctcaggcacgcattccctgctggtcgcacgggaatatttggagtggatatgcaggtctgctataaacatttaatattccgttccttttctcggttcaaaatgatcgcatttgttcctctcgcccgtcagcatatcgggatcgatatccccgtacacctggcaggaccgtatttccggcatgccgggcgcaaaggtcagcacgccgtagtgcacgcagttatagcacagcacgttttcctcgttgacataattctgctttaattggattcccaactgaattctctcctttatgattacatgttcgttatttttcatacccgtggtctttggaaaggtatacagctttttatagaagccgccggcaagataaaccggcacgagcgggttatgccccggaaaggccgctttccgctccaaaggaagggcagctctccggcgcatgctccgcatcgtgcctgaggcagtagcccttcgcgcagtccgcacaaaaataagaagacataggcggttccccgtttccatagaataactttattataccacgaaaaaagcggcggtgaacgctcccgccgcttaaaatatccgtaattacagcaattcgccgtactttcggataaacattttcttgagcgccgtcacgagcgccatatatgcgattaccgtaacgaacagcagcaggaaaaagctgcctggcatcgccatcatcccaagctcgcgccccacgatcgtgtagggaatgaccgtgcccacggcaatcccgatggatgtgagcagcgaaagctgccacgaggcgcggctccttataaacggtgtatgcggcgtgcggatcatgtggatgacgagcgtctgcgtccacagcgattccacaaaccaacccgcatggaacagcgcgacaaagccctcctgcgccgtttcgccaagcgtgtggtacgccccgccaaacaccatcgggcacagcaggaaatacattgcgaggtacgtcgtgatgtcgaacaccgagctcgtcggcccaatccataccatgaatttgctgatggaggaagcgtcccacgcgcggggcacgcgaaggtaatcctcgtccacattgtcccacggaacggcaaggcacgaaacgtcgtaaatcagattcagcaggagaatctgcacgggcatcatgggaaggaagggcagaaaagcgctcgccgccagcacggaaaacatgttcccaaagttggagctcgccgtcatcttaatatacttaatgatgttggcatacgttttgcgtccttcgatcacgccctgcccgagcaccgtcagatccttttcgagcaggataatgtctgcggattccttggcaacgtctaccgccgtatccaccgaaatgcccacgtccgcctccttcatggcgaccgcgtcgttgatgccgtcgccaaggaagcctaccgcgtgccccgaggcgcgcagagcacgcacgatccgcgccttttgctgtggggaaagcttggcgaacacatgcgtccgttccgccgccgcttcaagcgccgcgtcgtccatttcttccacgtccgcgccgagcaggacgtgctttgccgggatgcccacttggcggcagatatagcgtgtgaccgcatcgttatctcctgtcagcaccttcacgtccacgccgtaatctcgcagcatctcgagcgcccgcgctgtgctttccttgggcgggtcgaggaaagcaaggtagccaatcagcaccatatccgtttcatcatccacagagaacgcgccgcccgtatcctcgctcagtctatgcgcgattcccaagacccgcatgccatccgcgttatatccggcgacggtctcaagtatctcccgccgcacctcttcggtaagcgggatcacttcccctttgtattccgcatatgcgctcaccgcgagcatctcttcgatagcgcccttggtgatgatctgtgtttttccctttttatcagcgacaaccacgctcatgcggcggcggttgaaatcaaaaggaacctcgtccaccttgcggtaatcctccgcgagttccgccatccccacatcctgcgcatggttcatgacggcgacgtccatcaggttccgcaggcctgtctggtgatagctgttgagaaacgcgtggcgcagcacgcgcgcatcttttttgccatggatatcgagggaatattcgagcaccaccttgtcctgcgtgagcgttcccgttttatccgtgcacagcacatccatcgcgccgaaattctggatcgcacccagctgcttgacgatgaccttttccttcgacattgccaccgcgccccgcgcgaggtttgccgaaacgatcatgggcagcatctcgggcgtgaggcccacggccacggaaatggcgaagagaaacgcctgcatccagtcgcctttggtaaaaccgttcagaaacaacacgatgggcaccatcaccagcataaaacggatgagcacccacgaaacggagttcacgcccttttcaaagctggtcttgggtttgcgcgccgtcacctgccgcgcgagggaaccaagcaccgtatcgtcgcctacggcgatcacgatggccgccgccgacccgctgaccacgttgctgcccataaaggcgaggttgtcccgcccgagcacgtccggcccgcccgagcgcaccgtgcgtccaaatttttccaccggctcgctttcgcccgtgagggaggattggctcacaaacaggtctttcgcctgcagcacccgcaggtcggcgggaatcatatcgcccgccgcgaggcgcacgatatccccaacgacaatttcgtcaagcggaatttcctgttccatgcccccgcgcaccacggcggcagttgtctctaccagttctgaaagcctttccgccgcccggcccgagcgtgtttcctgcacaaactggagtgttcccgataccgcaaccatcgcaagcacgataataacggcaagcgcatcctgttcgcccggctcggcaagcactacgtccgtcacaaacgagatgacggcgagcaccagcagcacgatcgtaaacggatttaaaaacgccttgacaagccgttttaaaagggaatcgcctccgccgtaggtgatgcggttttccccgaagcgtccgcgcatatcccgtaccgcttcctgcgcatatcccccgtacgtattggaataccgtttcaaaacgctgtcctggcttttgcctgaagcgaggagcagcctttcttttacttcctgcgccctgcacgtttgcagggcaacgtttacttttttgttcattggtccttacctcctgtttgaagttccggacccggagaaacgagacgcagtgcgccgccctcctgggccctggtctggtttttggtccgccatgtccacgtttctcacttcctttcgcaatcaaatcatagaaacaaaaaatcccgccgaagcatgaacgcaacagcgggactgttcccacagaaacacacgaaaaaacgcgctaccgttcaagcttcagcatcgcagggcaatgaaattgcattagtctatgccttggtttcgacataaactgctgaccctctcatagtgtctccactattttgcggcagcaatccgtatccctgcggtaacctcgcctaccgaaatcgaactattcatttccggtttccagtatacccgcgcgccgcgccgttgtcaactttagtcccgataataccggaggattacgcttgcaggcacagcacgtttgcggtaagatatccatatatcaattaaccacaacttgcggaggcggaacatgaaatttgcgaataaaatgaaagtgttcgatttgaatattttttccaaactggaggaaaagcgcgcggaactcctccggcggggcatggaggtcatcaacctttcggtgggtacgcccgatttcaggccggatgaccacgtaatcgcggcgctgaaagaagcggcgggcatagcgggtaacttcaaatattcccttgccgatatccccgaactgatccaggcggtgatcgcgtggtacggccgccgctacggcgtttcccttgagccgcggcaggtgatgtccgtctatggtacgcaggagggcatggcgcatgtagcgctcccgatctgcaatcccggcgaccttgtgatcgcgcccgacccgtgctatccggtgtttatgtttggcccgcggatggcggaggcggaaatttattatacgccgctaaaaaaggaaaataattttctgattgattttgacagcatccccgaagatgttgcccggcgggcaaagatgatcgtcgtttcttatcccaataacccggtgacggcggtcgcggattacgccttttatgaaaagctcgtctcatgggcaaaaaagtatggcgtgatcgtgatacacgacaacgcatattccgagcttgtgatggacagcgaaccggggatgtcgttccttgccgttccgggagcgatggatgtgggaatcgagtttaattccctctccaaatcctacaacctgaccgggctgcggatctcttttgctatgggcaatacggaaatcatccgcaacttccgctgcctgcgttcacagatcgattatggcatttctttcccggtgcaaaaggcggctattgcggcattaaacgggccccaggatattcttgaacgcaaccgcaagggataccgcgagcgcagggacgcgctgtgcggcggcctgcggagcatcggctgggacgttcccgattccccgggtaccatgttcgtatgggcgccgctgccaaagggctatgaaaagtcgtgggagttcgcgcttgagctaatggataaaacgggagtgatctgcacgcccggcgaaagctttggccctgctggcgaagggttcgtgcggcttgcactggtggcagatgtgcccaccatcgagcgtgcggtgtgcctgatccgtgaaagcggaatgatccgatgagttatggatggctcggcggttatttgctccagaaagcgggcgtgaccacagactaccaacccgaatggcaagccacccgttatttcgtaggcggaaaaatgtttgccatgcaaggcggcgacaggaacaaaagacctatttttacgatgaaactcgagccttcgctgggggatttcctgcgaaggcagtatcccggcgcggtcgttcccggctattatatgaataaggtgcattggaattcgctgtaccttgaaagccgcgtccccgaagaaactgtgcgcgaaatggcagataaagcgtatgaagccggcctttgcgcattatcgaaaaaaaaacggagcgagatcgaaaacgggaaggaatagaatatgctgatcgattttgaacaactggacgaaacggagatcaaaaacttctatggcggcacgcaatccacttatgcgcggatgtttgcggacgaaagcaaccgtatcatgcgcggacggcttgcgcccggcgcgtcgatcggtccgcacacccatgaaacgggcagtgaaattattttcatcctttcgggaacaggaaaggcgttttgcggcggagccacggaagccctgacgcccggtatgtgccactattgcccgaagggacatacgcacagccttacggcggacggcgccgaggcgttggtcttttttgcagtcgtcccgcagcaataacaagcaaaagaggcgcttccgcgcctctttttttgtcttttttccgcgtgtgaatccgttatgccggcatcaggctgccgccgcccgcgagggcgattgtctgtgcgccgagccattcgtttcctgccgcgtccgcatcgtaatacaggttatgccctccgctcacaatatttgcgcacgtctcgtccgcatttgtgaggaccgtcacatagctgtctccggtcagcgtccatgcgctgtccgcatcgagggataccgccgccgcctgcgcggtgttctccgtgttgaccgcgcctgtaaaggtgctgccctgcgtaagtgaaagcgcaaaggtgctgatctcgtcgcacgtcacgtcgccttcaaaaacctggtttatacccgtcagggtaaactgcccgccatttgagccgggcgtgccccagttattggtctcgttgcccgccacattcgcaaggacgccgcttgtgaagacgagttccgtattttcaaagaacgcctccgcctgcgtattggtcacatagatcatcgggccgtccgacgtcgtcgtgagcctgctgtccgccgcttcaaagcgtgcggtcccctctgccgcgtcgccggaggtgctctgatagagcatgataccgttttcccccgccccggtgaggtccgtatccgtcatggtgatggagttctttccttccaccactgccgcctggctgcctgccgccgttcccgtgaggctatttaccgtgatgtcccccgtcgaatagatgcatgggctgccgtcgcccgccgcgaagaccgttccggtgtttaccgtgatggttccttcgccgcggtctgtagcgatgggcgcacaatgcgcaccttgcgtcgtaatatctacatttgtggcgttgaccgttccgccataggtggcgtcaaggccgcgggaggaattcccggtcgtatggatggtgacgttatccgccgtgaccgtggagtcctcacccgttgcaaagatggcgttcgagccttccgccgaggaagtcaataccgtatccgaaatctcggctgtgctgccgcctgccgccgcgaatacggcgtttaccgcataaaaattactttcatccgtactcgacgtatcgcccgttttatcgagcgtcccattttcgaggatcaggctgccgccgttttttacgagtacggtattttcgtctgcagacgaggaagcaatttcttcgccgtccgaggtcccgctggtgccgtccaccgtaaatacgcccgcaagctcgatacttcccgtctccgagccgctcaaatccccgccggggccgcccgcgccgccggcatttataatctcaagggtcgtgggaacaaaggattcgctttcgcccgatccttccatcttaacaaccgtaccttccgtaaggccggcgggcgacgcctctgtctcgctgccgccgtcctgttttgtgatggtgaccgcagtaaggtcgacggtgatttccgttccgtcttcatccgcggtaaagccgcccgccccgccggggccgccttcgcccagatcaggtggtgtgccgccgtttcctgcgtcttcggacggcgcttcaccgcttggcatatccggcgcctcccccgacggcatttctccgctttccagatcgggcggtgtgccgccactcattccgcctgtcaccgtcccgagggcaatcgtcgcttcattcccgcttaccgcggttaccttcccatatatcgcgtcatcctgaacctgcgcgcccgtttcctccgccggggcagcggacgaagtctccgccgcctgctgcgcacaggcggtaaaccccatcgccagaaccgcgcacagcaggaccgttaatatttttttcataccagttgttgctcctttcttggtctggtcccattatggaagcgtaacgtgaaggctgtgtggtgaaaggatgaaaaatctgtaaacgccaaaaaacgcccgcggggaaattccccgtgggcgttttgcgcataatttaccattcttccgtatacatatggatcggataggagaggtattccagcggatcaagctggtcgaccgtcacatatcctgccggtgcgttcaggattgtcggaatacggttcacaacggtcgcgcaggtgtgctccactgtcgctggtttgaccacgtgaaactccgtatcaggttcgccgacaatcttccagtcgcacatatcgccgtcgtccggcccgtataccttgccaatacactgggtctcgatcaccgggccctggtgcgtctgcgtcgtgacgaccgcgctcattccgatacagttgcccttcgggatcgtctccccggtggtttcagaatacaggtctttaccgtaaaaatacggtacgctcttttgcgtctgggatttgatcgtccagcccattttggcgcacagcgcctcgttggaattccacacataactcggttcgagaacttccgggtgggccagttgcttttcaaattcttccggtgtgagtcctacgccgtgcgcctgcgcgagcgcgagtccgtaatcctccacgttatagctgaccgctccttcgatgcggtctatagtatggacgccgcccgcaacgcccgcgatcatgttcacccaatagatatcctgcatccccgagcccacaatagtgcagcccgtttccttggcgaggacgtccagcttattcgtaagggcgggcgaggtcgtccacggatagatcgcttcttcacatgtcgtcactacgttgatgccgcgcgcggcgcatttttcgatatgcggatacatatcgtccatgaagctgaacagtgtaagaaccgcaatatccgcatcacattcgtctaggacagcatccgcgtcactgcggatcggaacgccgaggcgcacgccaaggcctgcccattcccctacgtccatgccaacgatgtctggattcacatcgaccgcgcccacgatatccgcgcccttctcatacaaataccgaaccgtatactttgccatttttccgcagccatattgtacggcacgaattttttgctgatacatattttctccctcttttcaaaaatttccaccgatgtccgcttgtgttgttttccccctggatactatcaatataccacccataagacacctcaaacctttttttaatcaaaagcgcccggcgggatcgccgggcgctgcttttcactttagctggaactgcggatcgcttcaagcggactcatcttcgttgccttccatgcaggataaatgccggacacaatgccgacgcctacggcgatcgcaatcgcgccgaggctgagccaccacgggatggaaagctgtaccccgttctggaaatacatgccgaggaagctgatctcgctgccgccgaaatttgcggccgcgccgaagatatagctgaccccgaggccgatcagccctcctataaggccgatcattgccgcctccacgaggaacatcaggttgatcttgcgaatggaaaggccgataaccttcattacgccgatctcccgcgcccgttcaaggatgctcgcgagcatggtattggcgataccgatcgccgataccagcagggagatgaggccgatggcgatgagctgcgactgctggcgcgcctgttcctcctgcatctgggtgatccattcggtggggctgtaggcctggaatcccatttccttgaccgccttgaggatgtcttccaccgcgtcaacatccaccgcgttcacatagccctgcgaatattgtccttctttgattcctgcctggtccatcagcttgcggttttcgcggataagcatattggcggcgggaatactcatatagatattatagctctcctgactgtccgactgcttaagaatgcccgtaatttttccgcggtattccttgggcgccggctggtcaggggtggatgggtctggattttcgatcaggtatccgctgcccgggtaatacttcacgttcgtccctacccagtctacatccggcccggccggttcctggtattcgccgtcgtcggccacggcgaccgcgtagccgccagccatcatcacgccgcccatcatgcctccggaggcattcgggtcctggaaatactgccgggcgttcgcgcccacgataagctccacgttagggctgtccgagaagacatttccctccatgaatttaaaatccatagtttgcgggtcaaccgcataaatataggtatccgccttatattttcccatcacaatatacgaggggatgctcatcaggccgctcgcgtttttcacccccggaatggcccgtatctggttcagcttggcatccgtaagcttggcgttttcccccgagcccatgggggatatctcgatccgcgtaaggtccgtactctgcatgatgctctggttgaactgctcaaggttcccgagaccgagcgccaccatgataacaatgcacgccgttccgataatcacgccgaggacggtcagtatggtccgcatcttgcgccgccacagattggatgccgcaagaagaacaatatcaataaatgtcatcgtcttcgaggtcctccgaaagctcctgcgcgcgtttttttcttttcctttttaccacaattacaatggccacggctgccgcagcgcctgcggtgatcccccagccccaccacgggaaacctgctggctcctccggcgggagctcttcgccgggatccatgccgccataatccggcataggcgtgaggactgtttcaaccggcaccttcatctcgtattcttcgccgtactcgtcttcataagtgacgacaaaatttccttccaccggaccgggctggacggcatcttccgcgcctgcgccgcctacagcctgcaccgtgccgctttcccccgatacaacaatcgagtccggtccatccgcaccgccggttattgcgccgtccgccgcgggagccacttcggcattcccggtttccgcgccgctcatgccgcccatccccgcattcgggtcctgggcaacggacgcatagatatccgccgtcttcgccgtgccggattccatatttccaagaaaagcgctcgattccggcgtaagaccgggaacgtcaagcacgaccgttacattataaagggtgttttttcccttgttgtataaattgaggctcgcggaggtggtatcgcccatatagacttccgatgggaatttcggcggatcatattcaagacggatcttctggtgcacctccacgctgatctcatccgccgccgtaagctgcgccgcctggctgtcttcgtaggcgatggcgatatcgatcttctgcggccccgctttggcgtcggcgcgcgcttccatcgtgaagctgaaatccgccgttttcttcgggccgatcttttcaatatacgccgtattggtattgtcgccgggcatcagatcggtcgtctggcttttgaaggtgactgtgatgtttttgacgctcgtcgatttgctcgtgttggtaagcgtcacctttacggtaaacttttcacccgcgttgaccggatcgggactgatctcgtaattgctgatgatgaccttgggctgagaactcactccgctccccccgccaccgccgcccgcgccgggatcgatccccgggtctgttcccgggtctgttcccgggtcttccgtcggctgaccggacggctccccacttggttcggccgtcggctcagaggggtcttgcccgtccgttaccttgacgaataccgtaaactcctgcgttttaacagtgccgtccataagcgggtatttcgcggtgacgacaaccggatagttcccattcaccctgttttccgcaagcggcaggctgaggtccaccaaataagactcctttgttttcccgtcggccagcttattttccttaagggatacggccgtatcgtaattattgaatataaagggagcggtcttgggatcgccgaggccaaccgaaatattgacctgttccccatttttcacctgttctgttcccgggccggggaccagcggaaggagaatgcgcgccgttcccccggatacggcggggctatatccctcctgataggaggcgttcatgcccccgtattgacttttgccgtcgatccggagcgccgttccgcgcatatccgcagcaaatgcggttggcagcgcaaacgaaaacgcgagtataacgatgagtgcgataattgtgatccgtttcttcatttttcctctccctgtattcctaattccgcctgtatgatctcttcggtacttatttcggcaggtccgtgcgtttcgcgtttcgccactttcccgtctatgatatgaataacctggtcggcatattccgccttggctggatcgtgcgtcacgaacaggagggtcgcgccgcgtttttttgcctgtccgcacataatgtccataatctgttccgcggtcaccgaatcgaggttgcccgtcggttcgtccgcaaagataatctccggctttgcgataatggcgcgcgcgatcgatacgcgttgctgctggccgcctgacagctggtttggaagatttttaagctgctgcctgaggcccatttccacaagcagtttttttgccgcttccatgcgcctggcgcgcggcacgccccggaacatcaagggcagcgccacgttttccaccgccgtcatggtgggcatcaggttgaacgattggaagacgaagccgatatgcttcaaacggaaatccaccaattcgctttcattcattttataagtcggttttttcttgataaaaatcctgcccgcggtcggatgttcaagccctgcaagcagggaaagcagcgtcgattttccgctgcccgaggtgccgagaatcgcgcacacctctccgggcatcacatcaatgtccacaccgtccagtgcatgtatttttgcactgcccatgcggtatatttttttcagattcctggctgcaatgatcggttccaaagacttcctccaaaaatggcgtctttcgggcataaaaaagccctgcacgaagtgaaggggaaacggcaaagatcccacccctaacctacgtctttcattatagcataaagaatctttccgttgggcggcactttatgaataaattcttacaaataatatggttttttaaaaattattatcgggacggcggaaggccgcgaaccgtcctccgcagaatatagagaagggaaacgcggatgcgtttcccttctctaattttatagtcctgcggtttccgttctaagtatacggcaggctcggttctcaagcgaacggcgctgtttcagccctcgatgatcttgacgaacgattggtactgcgcagcccattccgccgtatcccggggggtatacgtcttcggcgcacaggacgcggccaccacgcggcgcgcctctttgatgtccttgatttcacccgcggcaatgagctgtactacgatgttaccaagcccggttgcctcgtccggtccggcaattacggtcatgcctgtcgcattggccgtcatctggcacagaagcgcgctctttgtgccgcccccaaggatatgcaccgtaccgtattttttgcccgtgcattccgcgaggcgtttgatgctgtaatgaaacttcatggccaggctttcgtcgatgcagcggatgatttcgccttccgtctgcggaacaggctgccccgtcttttcgcagtaggcgcggatacgcctgggcaggtttccaggctttccaaattccgggctgtccacatcgatcaggctacggaacggcgtgcattctttcgccatctgctccagctctccaaagccgaactccttgccctcgcggatccactggcggcgggactcctggatcggccacgtacccattatatttttcaggaaacggtaagtgccttccaccccgccctcgttcgcgaagttgtatcccgctgccttttcgttgatgcagggttcgtgcagctcggtgccaagcaggctccatgtaccgcagctgatgaaaataaaatcatcttcctgcgtgggggtcgccgcgaccgccgccgcagtgtcgtggccggcagtacacatcactttggctttgggggcgccaagttcttcgcagatgtcgtcgcgcagcaggccgcactcggttcccggctggacgatatcacataatttttcgcgcagaatgcccgaaagctccagcaccttttcactccagtccctgcttttcgcatccagcatttcagatgtggacgcaatggtgtattccgtatgcatttcccccgtaaggaaatagttgtaaagatccggcgtaaagagtatttttttcgtcgccgccagaagctcgggcttctgctccttcaggtaaagcagttggtaaagcgtgttgatggctagatgctgcaggcccgccgtctgatacagctcgtccggatcaatccgcttcatgaattcctcaaacggctgttccgaccgcccgtcgcggtaatgaacagggttctggacaagctggccgtcttccccgatcaagccaaaatcgacgccccatgtgtcgatgccgatcatatcgaagcctcccgcaagcgccgccttgctgatgccctgcttgatattgtaaaacaggcgcagcgcatcccagaaaagcgtcccgttcagcgaaaccggatcattggtgaagcggtggagttcttccattgtaatttttccatccgcatactgggcgatcattgcacggccgctggaagcgccgaaatcgaatgctaaaattctgctcatgctctttcccctttactatttctattatattaactatactgaaaataagaatcggaatcaatgaagaaaacaacaaatttttgtaaattttcaacactctttgtttggatatgcggtttttttgtttttcccggaattgatgtcacgtttcgtttgtgagataataaaaatataatcatcacccagcctgagaggacggaggaaagatcatggactatgtaaagctcggcagaacggatctgaagataagccggatggtaatgggcggagacgtgcgcacaccccgcgaggaatttgccgccgcgctgcagcttgcggtggatcatggcgtgaacctcatcgataccgcgcccgcctacgggaacagcgaggaggtccttggcacgattctcccggagatcaggggcgagttgtttgtatctactaaattcagcaacgacccgcagccttttttgccgcaggaccgggactgcctgatgcgtgccgtggaaaacagcctctcccgcttgaaacgcgataagatcgatatctggatggtgcatgagcccgaccgtccgtatcaatacgactggtgggaacgcccgcaggaccttaatcatcctgaagcgtattatgggccggtcatggatgtgctgtccgacctgaaaagccaaggcgttatcaaatatacgggcatcggcgggacgacggcatatgagatcgtgccgatcatcgaaagcggctttttcgatgtgatactgactgccttcaactacagccttttgtggcaggaggcggccatcgaggtaatccccgcggcgaaaaagcagaatatggggattttgcttggctccgcgctccagcagggcgcgctcgcgaagcgctacgacgaacaggtaagggcaaagccggcatggctttcaaagccccgccagcagcaatacctgaaattatacgagctgtgcgacgatttgaagatcgatatcgcagaccttgcgatgcggtttgcattttcaaatccggatatccacgccgtcgtaacgggcgcgggcaaggtgaagaatgtgcagcggaaccttgagtcgtaccacaggggcccgctgccgcaggatgtgctcaggcgtatcggtgaaatttaccggatggtacccttccgcccattcgaggaatcgtttttcatgccctttacgcgcccctataaagggccgcgggcggtgcactgaacggcttcggctttccgcacatccgccaaataatttttgtattaaaaaaggacaggcaaccgcccgtccttttttgatcccggtttatttcttcttcagctcgtcgtccgtaatctgcaggctcctgcgtacgatcttcttggaaaggaacttgtccgcgcgtttttccacaatgcgttcaaagccccgcatcatgaacggcgcgaccgccgtgaaaacacacactacaacggcctgcggaaggctgattggcgccacatcgaaaaagcccctgaggaaaatgatgcacaggatgaacaggccaatggcgctgccgaggatcaccttgcgcgccgtggtaaacggcatgctgaccttagctaccacccacataccgaccgcaaccgccatgagcatgcacatcgtggagaccgccgccggggtgtattggaagattcccgcaagcacgttgaccgcaaggattccgataataacggaaagccctccgggcaatgatttttttaaaatattaatcaggaaatgctccttgatcggcgcaaaattcggctccaaagcaaggaaaaacgccgggaagccaatggtcacaaaactgattagcgtcatctgcaggggcgtaaacggataactgctgtcgagcaggattaccgtcgcgaacgcaaggagcaccgcatacaccgttttggtaataaacagagtggccacgcgttctatgttgttgattaccttgcgcccttcatttacaatatcgggcatcgtcgcaaaattagaatcgagcagcacaaggttggcgatatttttagccgcgtcgctgcccgacgccatagcaatgctgcaatcggattccttcagggccagcacgtcgtttacgccgtcgcccgccatggcgaccgtatgacccttgcgtttcagcgcggcaatcaattcctttttctgggaaggcgttacccgcccaaacacgctgtacttttcggcagccgcctcaatatcctccttcgttttgagcagggtggcatccaccgcttcataattttttacgcccgcgcgtttggcgatcgcgccggccgtgaccggactgtccccggatatgatcttaagctctacctgctgcttctcaaaaaattcaagcgtctttttcgcatccgcccgaatccggtcggaaatgagcaggaacgcgatggggcgcattcccccggggaccttgttatccagcacgtcggtggcgtcgctgtgcgcaagcaccagcacccggcttccttgtttcgcgtatttttccgcgtcgaggcccgcatacccgttgggaaaaataaactcgaaggccccgaggaaataggtcccttccccttcaaagcttacgccgctgtatttacgcgccgaagaaaatggcacgatggtttttacttcatggtcaaagctcttgccgaatttttccactacggcatggaaagtcgcgttatcgtcctgaagcgctccggccatattggagaggatcctgtccaagtcttttgcagcgcctacgggaatgacttcctccacatgcatctttccctcggtgatcgttcccgtcttgtcaaggcacaggatatctacacgcgcgagcgtctcgatgcagtagaggtcctgcacaagcgtctgctttgtcgcgaggatcacggcgctggttgcaagggaaatactggtgagcaggataaggccttcagggatcatgccaataagggcccccaccgttttgaccgtattatccggtatgggcaggcccaccacaagcccctgtttcagaaacagcagaatacccaccggcacgatgatgatgctgataattttaaggatgcggttgagggaattgcgcagctcggacgtacgctttttagatgccttcgcatcataggaaattttatttgcatagttttcaattcccacgcgctccacacgcgcgtaagcgttgcccgatacgataaagctgcccgaataaagaaagtcgcccgggcccttggccacaacgtcggattcgcccgtaatcagggactcgttgacctccaccgatccttcaagcatcaccccgtccgcacatacctggttgccgggccgaagctgcatcacatcgtcaaggacgatatccgcaacgccgatctccttttcggctccgttccgtaccaccgtgaccttggccgccacgatcaccgagagcttatcgagcgttttcttggttacgatctcctgtgcaatcccaatgacaaggttccccacgacaacgagcaggaaaacaagttccttgatgtagcccgtcatcacgataaggaccgtgaacaccatattcagtatattaaaaaaggttacaaggttatccttaaaaatctgccggtacgattttgtcgtattcgtattatacgcatttgtgagacccgcatcaatacggcttttgacctgtccgtccgtaagccccgtgcggcagtccgaatcatagcgctgttgcccgtcgtccatgtcgttccttccccgtcattacatagtgactttattatatcatatttaccctatgctccaatgattatccgccaaaatttataaattcctaacaaaaacgacggatttcttcatccgccgtttcaaaagtcttaagaattcccttatttcgtgaggaaccggtattccgttacgtcgtggtaggtctttcccttctgcaggatgcaggaaggaaattcatcgtggtgcacgctgtccgggaaaagctgcgtctcaaagcaataggccgtacgcgggccgtattgcactccgttcttccccttcatctccggcacgaagttcgccgtatagagctgcatgcccggtttgtccgtatagacctccatcacgcggccgctctgcgggtcttcaacccgcgccgcacgccggaagcccgcgccccacaaaacaaagttgtggtcgtatcccccgcacagcttcatctgcgggaatggatcttcgatccgctcgccgatcaggtgcggatgcgtgaaatcgagcggagtgcccgcaacctcggcaatctctcccgtggggatcaggttgccgtccaccggcgtatattccccggcgtcgatggtcagcacatggtcgctgatctcgccctccccccgcaggttgaaataagaatgatttgtgagggacaatatggtgtcctcatccgattctgcaaaatattcgaggcgcactgcattatcgtccgtaagggtcatttcaatgcgcacatccaccgcgcccgggaagccgccttccccgtccggactgtgataggaaagggtcagcatattgccgtctgccgtaccgtcccacaccttgcggttaaagctgttgtctcctccatgaagaagatttaccccgttttcgttgcacgggatggcgtaatcctttccgcccaccgtgaaccggccgtttgcgatccggttggcataccgcccgactgttgcgccaaaaaagggatggccgccaaaatactcctccggcgtttcaaagccgagcactacatccgccctattgccgtctgcgtccggcatttcgaccgacataatcgtcccgccataattcgtgaccttcatgcatccgccggcttcactcgaaaatgtataaacaaaaatatccttaccgtctttactgccagttttttgagtttcaatcatgatctttaccgcccttttgatttgctattattattctacatcaaaagcggcttttttcctatccgttatcaatcaattttttgtgaaattttcttttgcaatatgaaggaggtgtgctataatagttagcagtggaggcatagctcagttggtcagagtacctgcttcacatgtaggg

SEQ ID NO: 2 - DNA, 978 bp, Christensenella minuta
  CP029256.1:1933575-1934552 BSH gene
atgtgtacagcaataacgtattatacaaaggatcactattttggaagaaatctggatctggaattttcttataatgaaacagtaacggttacaccaaaatattatccgtttcattttcgtaatggaaaagtgctcaatcatcattatgcaatgatagggatggcttatatagttgatgactttccgctttactacgatgcaacaaatgaaaagggtctcagtatggcaggactgaacttcccggataatgcggactataaagaagtgaaggaaggatacgataatattgctccctttgaatttattccatggatactcggtcaatgtgcaagtgtgagtgaagcaagaattctcttagaacagattaacttggtaaatttgaactttagtgaagagctgccgctttctccattacattggatgatttctgaccagcgagattccattgtagtagaatcaacaaaagatggtttgaaagttttcgaaaaccctgtaggagttctgacaaataatcctacctttgactatcagatgtttaatctcaataattatatgcatttatcgaaagaaccccctgcaaatacatttgctgccgaattggaacttgaacagtatagccggggtatgggggcgataggccttcccggagatttatcatccgcttcgagattcgtgaaagcagcgtttacaaagatgaactcggtttccggtgattcggaatcggaaagtatcagccagttttttcacattcttggctcggtagagcagcaacgaggctgcgtacatcttggtgaagataaatatgaaataacaatttattcttcctgctgtaacatggacaagggaatttattactatacaacttatgaaaacaaccagatcacagcagttgatatgtataaagaaaatctggacggaaacactataataagctatccgcttatgaaagaacagcagattaactatcggaattactaa

SEQ ID NO: 3 - DNA, 129 bp, Christensenella minuta
ctcggtcaatgtgcaagtgtgagtgaagcaagaattctcttagaacagattaacttggtaaatttgaactttagtgaagagctgccgctttctccattacattggatgatttctgaccagcgagattcc

SEQ ID NO: 4 - DNA, 121 bp, Christensenella minuta
aagaaccccctgcaaatacatttgctgccgaattggaacttgaacagtatagccggggtatgggggcgataggccttcccggagatttatcatccgcttcgagattcgtgaaagcagcgtt

SEQ ID NO: 5 - DNA, 86 bp, Christensenella minuta
tgctccctttgaatttattccatggatactcggtcaatgtgcaagtgtgagtgaagcaagaattctcttagaacagattaacttgg

SEQ ID NO: 6 - DNA, 20 bp, Christensenella minuta
  BSH_qPCR_F2
ctcggtcaatgtgcaagtgt

SEQ ID NO: 7 - DNA, 20 bp, Christensenella minuta
  BSH_qPCR_R2
ggaatctcgctggtcagaaa

SEQ ID NO: 8 - DNA, 20 bp, Christensenella minuta
  BSH_qPCR_F3
aagaaccccctgcaaataca

SEQ ID NO: 9 - DNA, 20 bp, Christensenella minuta
  BSH_qPCR_R3
aacgctgctttcacgaatct

SEQ ID NO: 10 - DNA, 21 bp, Christensenella minuta
  BSH_qPCR_F6
tgctccctttgaatttattcc

SEQ ID NO: 11 - DNA, 23 bp, Christensenella minuta
  BSH_qPCR_R6
ccaagttaatctgttctaagaga

SEQ ID NO: 12 - DNA, 26 bp, Christensenella minuta
  BSH_qPCR_probe2
agtgaagagctgccgctttctccatt

SEQ ID NO: 13 - DNA, 27 bp, Christensenella minuta
  BSH_qPCR_probe3
actgttcaagttccaattcggcagcaa

SEQ ID NO: 14 - DNA, 27 bp, Christensenella minuta
  BSH_qPCR_probe6
cacacttgcacattgaccgagtatcca